European Patent Specification EP 4 338 586 B1, published March 18, 2026. Title: ELITE EVENT CANOLA NS-B50027-4. Applicant: Nuseed Nutritional Australia Pty Ltd. Application EP 24151478.5, filed June 16, 2017. The sequence listing filed with the application follows.

SEQUENCE LISTING (66 sequences)

SEQ ID NO: 1 - DNA, 44 bp, synthetic construct
  misc_feature 1..44: note = KASP primer
  source 1..44: mol_type = other DNA
gaaggtgaccaagttcatgctccaagcaccgtagtaagagagca

SEQ ID NO: 2 - DNA, 26 bp, synthetic construct
  misc_feature 1..26: note = KASP primer
  source 1..26: mol_type = other DNA
gctaagaagtggggactcaactacaa

SEQ ID NO: 3 - DNA, 41 bp, synthetic construct
  misc_feature 1..41: note = KASP primer
  source 1..41: mol_type = other DNA
gaaggtgaccaagttcatgctgctcttgctggaactcttgg

SEQ ID NO: 4 - DNA, 26 bp, synthetic construct
  misc_feature 1..26: note = KASP primer
  source 1..26: mol_type = other DNA
gggttagccacattgtaggtaacgta

SEQ ID NO: 5 - DNA, 44 bp, synthetic construct
  misc_feature 1..44: note = KASP primer
  source 1..44: mol_type = other DNA
gaaggtgaccaagttcatgcttaagagacaccctggtggaaaga

SEQ ID NO: 6 - DNA, 28 bp, synthetic construct
  misc_feature 1..28: note = KASP primer
  source 1..28: mol_type = other DNA
tagcatcagttccaacttggtaagcaat

SEQ ID NO: 7 - DNA, 44 bp, synthetic construct
  misc_feature 1..44: note = KASP primer
  source 1..44: mol_type = other DNA
gaaggtgaccaagttcatgctgaacacgtaagcagaccaagcag

SEQ ID NO: 8 - DNA, 25 bp, synthetic construct
  misc_feature 1..25: note = KASP primer
  source 1..25: mol_type = other DNA
ccctcttctccctaacgaattcctt

SEQ ID NO: 9 - DNA, 44 bp, synthetic construct
  misc_feature 1..44: note = KASP primer
  source 1..44: mol_type = other DNA
gaaggtgaccaagttcatgctgaggaacctgttgctgctgatga

SEQ ID NO: 10 - DNA, 26 bp, synthetic construct
  misc_feature 1..26: note = KASP primer
  source 1..26: mol_type = other DNA
gcgatcctagcacaaagttgaaggta

SEQ ID NO: 11 - DNA, 44 bp, synthetic construct
  misc_feature 1..44: note = KASP primer
  source 1..44: mol_type = other DNA
gaaggtgaccaagttcatgctggatggatcgcttacctcttcgt

SEQ ID NO: 12 - DNA, 25 bp, synthetic construct
  misc_feature 1..25: note = KASP primer
  source 1..25: mol_type = other DNA
cagggtaaggttgtcctgtaacgtt

SEQ ID NO: 13 - DNA, 42 bp, synthetic construct
  misc_feature 1..42: note = KASP primer
  source 1..42: mol_type = other DNA
gaaggtgaccaagttcatgctctattggatggggactcaagc

SEQ ID NO: 14 - DNA, 26 bp, synthetic construct
  misc_feature 1..26: note = KASP primer
  source 1..26: mol_type = other DNA
gggagatccttagtagcagaagagat

SEQ ID NO: 15 - DNA, 44 bp, synthetic construct
  misc_feature 1..44: note = KASP primer
  source 1..44: mol_type = other DNA
gaaggtgaccaagttcatgctcctgagaggcgtcctgttgaaat

SEQ ID NO: 16 - DNA, 25 bp, synthetic construct
  misc_feature 1..25: note = KASP primer
  source 1..25: mol_type = other DNA
aacagcagccatatcagcagcagta

SEQ ID NO: 17 - DNA, 45 bp, synthetic construct
  misc_feature 1..45: note = KASP primer
  source 1..45: mol_type = other DNA
gaaggtgaccaagttcatgcttgttcttgggtgggtctgtccttc

SEQ ID NO: 18 - DNA, 46 bp, synthetic construct
  misc_feature 1..46: note = KASP primer
  source 1..46: mol_type = other DNA
gaaggtcggagtcaacggattgtgttcttgggtgggtctgtcctta

SEQ ID NO: 19 - DNA, 25 bp, synthetic construct
  misc_feature 1..25: note = KASP primer
  source 1..25: mol_type = other DNA
atccactagcagattgtcgtttccc

SEQ ID NO: 20 - DNA, 22 bp, synthetic construct
  misc_feature 1..22: note = KASP primer
  source 1..22: mol_type = other DNA
gttggctaaggtcacggtggag

SEQ ID NO: 21 - DNA, 48 bp, synthetic construct
  misc_feature 1..48: note = KASP primer
  source 1..48: mol_type = other DNA
gaaggtgaccaagttcatgctccgccttcagtttaaactatcagtgtt

SEQ ID NO: 22 - DNA, 41 bp, synthetic construct
  misc_feature 1..41: note = KASP primer
  source 1..41: mol_type = other DNA
gaaggtcggagtcaacggattggtcacggtggaggtcacca

SEQ ID NO: 23 - DNA, 22 bp, synthetic construct
  misc_feature 1..22: note = KASP primer
  source 1..22: mol_type = other DNA
ggtgtgttcttgggtgggtctg

SEQ ID NO: 24 - DNA, 49 bp, synthetic construct
  misc_feature 1..49: note = KASP primer
  source 1..49: mol_type = other DNA
gaaggtgaccaagttcatgctacttttttttcaactgttggctaaggta

SEQ ID NO: 25 - DNA, 49 bp, synthetic construct
  misc_feature 1..49: note = KASP primer
  source 1..49: mol_type = other DNA
gaaggtcggagtcaacggattacttttttttcaactgttggctaaggtc

SEQ ID NO: 26 - DNA, 21 bp, synthetic construct
  misc_feature 1..21: note = KASP primer
  source 1..21: mol_type = other DNA
gtgtgttcttgggtgggtctg

SEQ ID NO: 27 - DNA, 21 bp, synthetic construct
  misc_feature 1..21: note = KASP primer
  source 1..21: mol_type = other DNA
gtcgtttcccgccttcagttt

SEQ ID NO: 28 - DNA, 46 bp, synthetic construct
  misc_feature 1..46: note = KASP primer
  source 1..46: mol_type = other DNA
gaaggtgaccaagttcatgctaaactatcagtgtttgaacacctcc

SEQ ID NO: 29 - DNA, 44 bp, synthetic construct
  misc_feature 1..44: note = KASP primer
  source 1..44: mol_type = other DNA
gaaggtcggagtcaacggattacaacttgtcgtgctacacacct

SEQ ID NO: 30 - DNA, 22 bp, synthetic construct
  misc_feature 1..22: note = KASP primer
  source 1..22: mol_type = other DNA
ggttgtgtgaaaacgtgtgagc

SEQ ID NO: 31 - DNA, 51 bp, synthetic construct
  misc_feature 1..51: note = KASP primer
  source 1..51: mol_type = other DNA
gaaggtgaccaagttcatgctcttttagctaaataagaggttctgtatact

SEQ ID NO: 32 - DNA, 51 bp, synthetic construct
  misc_feature 1..51: note = KASP primer
  source 1..51: mol_type = other DNA
gaaggtcggagtcaacggattcttttagctaaataagaggttctgtataca

SEQ ID NO: 33 - DNA, 19 bp, synthetic construct
  misc_feature 1..19: note = KASP primer
  source 1..19: mol_type = other DNA
gattgtgattccgggcagt

SEQ ID NO: 34 - DNA, 21 bp, synthetic construct
  misc_feature 1..21: note = KASP primer
  source 1..21: mol_type = other DNA
gtgtgaaaacgtgtgagcaat

SEQ ID NO: 35 - DNA, 40 bp, synthetic construct
  misc_feature 1..40: note = KASP primer
  source 1..40: mol_type = other DNA
gaaggtgaccaagttcatgctttgtgattccgggcagtag

SEQ ID NO: 36 - DNA, 41 bp, synthetic construct
  misc_feature 1..41: note = KASP primer
  source 1..41: mol_type = other DNA
gaaggtcggagtcaacggatttgtgagcaattgttggaggt

SEQ ID NO: 37 - DNA, 31 bp, synthetic construct
  misc_feature 1..31: note = KASP primer
  source 1..31: mol_type = other DNA
tcttatcaacattaagaacataatcttttag

SEQ ID NO: 38 - DNA, 15 bp, synthetic construct
  misc_feature 1..15: note = Insertion deletion on Brassica chromosome A02
  source 1..15: mol_type = other DNA
gtagcacgacaagtt

SEQ ID NO: 39 - DNA, 20 bp, synthetic construct
  misc_feature 1..20: note = Insertion deletion Brassica chromosome A05
  source 1..20: mol_type = other DNA
cacggtggaggtcaccatgt

SEQ ID NO: 40 - DNA, 15004 bp, synthetic construct
  misc_feature 1..15004: note = Transgene insert and Brassica flanking regions
  source 1..15004: mol_type = other DNA
gagccttgagtgctactttgggaacaaaaacttggtttgatgctatcctagtctttttctcttttataaactattattagataaaaactaaaaaatagtatttatgagatttgtctttttttcacaatataaattattttaggtataaaaataaataatagaattagtattattagatatataaaatacatttaatttaattaataatataactgtaaagtataattaagttatacaatatctaataaatataaaaattgtattaaaatatgggaaaacaatattatattttaaagcgatcttactcgatctctctttgatcccaaagttttcattccttttaattatatttgttgcagaatattaaaaccagtgatttctggggtttgataggattaagacacgatcgcagagaaagtagaatcaatcgtggaagggaagggatattcgaaaccctaatttcgatcgtatccccatcttctacgaaagcatcgatcgacttttttctgattcagtgagagtttgaaatcaaagtttgattttttcgacctgatgggtttcttaaagaagttaacggggattttcgggttcgggcacaacgatggtgggcacggagctgctgcgagagacgaagatggtgaaggggataacactggatcagtctctgaggacggagataaacgccgggagggtaatcaggcaaggttccgtgaaaccggacttccaaggaggggttttggagttccggttcaagtagccgtcgaacggtctagtcctggtcctattcttcagccttgtgctgcttctgacggtggagttcaggtttgtctttctttcatggttgtgattttaactgtgtagaagtctagggactgaagaaattaatgagaatttgagggttgctagttttgattctgatcttgtaatgtggctacagtgttgtacttgtcttgttgcaggatcgttaaatccatttgtttggttccgatcatcctatgttagttggtaaaattggtcttgtgagtttgtttaagttgtttttgtgtcttcattcattttctaagcttagcattgatgaacagttgaatttagaatctttgttctaagcttaacattaatgaatatcgaatctttgttctactcagtcctttctttgtttttggttgtgatatgttctcgtttcaacgtagtttatgttcttcttgtgattggctttacattctgcacggtttccgctttagttaggtgtctgcattatagttagttcattgctatcttaaattctctgttcattcatctctatatatcaaattaaagagtggcagtgaagtttatgacaggacacgatatatgttttagcttgattagttgcggttaaagcaaaaagtttttgtttcactctgtctgctacagaacctgtaatttagaaatgatgatggatctcatgtcttaacggtttcgtattcatcatgagtcacgaggctgctatagagtttgaatcttaattggttctgttgttggggaaagacaataatccagtctttaagaagctagtggggttgattcatccccaagactattcgattgtccaaacgcattgatatgttttttttaatcaagtttttgttgatggcaataaactaacatcccagcatagttattgactcgacttagttttaccattagggactacgatggtactcaatgcggctaaggattgatgaagatggagatgttgcagatgagttcttggaagatgataactgtaagactttgcccagaaaatgcaaaacaaaagctgcaaaagtgagaggtttagtgatatcttctgatgggaaacttcagccattaatgcattgagcagtgaacaccaaggataaatatttactgattagtgtgtgattgaatcaaagaaaggttagaatctggttttcatttagccattcaatctcgatgtaaaatcggttagattctggttgttgatacttgagaacttgaaatgttttgtaactgtgaattttgttttgaaaatagacaagtgaatctgtttggggttgtgtgaaaacgtgtgagcaattgttggaggtgttcaaacactgatagtttaaactgaaggcgggaaacgacaatctgctagtggatctcccagtcacgacgttgtaaaacgggcgccccgcggaaagcttgcggccgcggtaccgcccgttcgactcagatcttccaaggcctcgtctccgagtccgctgcttctcgccgcgccgatcacttctccgccgccaacaaggcttgtagttaataggaatcattcagggattgtgattccgggcagtagtaattaataatatagtattagtatagataatatgtttcgtttgggatctttggaacgttgctctgttccttgttgttcattttaaagcttttgagggatagttgcagaactgttcggtgatgcttcatcctctcaagaactagatttgggtaaagaaacatccatgcatggatatggaatgttgttcttccgattggagattattttataaaatttaaaattcatgatttaaaaaaacacataaaaaccacaaaattcatgatttattgacaatacgatacaaaattagcaccaccggctactggctcattacacatttccccttcccctcattctcactttgtggctttattattattattattacatatattttaccgttattatttcacgtcacataagcttgttaattaatcattagtgagccttctcagcctttccgttaacgtagtagtgctgtcccaccttatcaaggttagagaaagtagccttccaagcaccgtagtaagagagcaccttgtagttgagtccccacttcttagcgaaaggaacgaatcttctgctaacctcaggctgtctgaattgaggcatatcagggaagaggtggtggataacctgacagttaaggtatcccataagccagttcacgtatcctctagaaggatcgatatcaacggtgtgatcaacagcgtagttaacccaagaaaggtgcttatcagatggaacaacagggaggtgagtatgagaagtagagaagtgagcgaaaaggtacatgtaagcgatccagtttccgaaagtgaaccaccagtaagcaacaggccaagagtatccagtagcaagcttgataacagcggttctaacaacatgagaaacgagcatccaagaagcctcttcgtagttcttcttacggagaacttgtctagggtggagaacgtagatccagaaagcttgaacaagaagtccagaggtaacaggaacgaaagtccaagcttgaagtctagcccaagctctagagaatcctctaggtctgttatcctcaacagcagtgttgaagaaagccacagcaggagtggtatcaagatccatatcgtgtctaaccttttgaggggtagcatggtgcttgttatgcatctggttccacatctcaccagaagtagaaagtccgaatccacaagtcatagcctgaagtctcttgtccacgtaaacagatccggtaagagagttatgtccaccctcatgttgaacccatccacatctagctccgaagaaagcaccgtaaacaacagaagcaatgatagggtatccagcgtacataagagcagttccaagagcgaatgtagcaagaagctcgagaagtctgtaagccacatgggtgatagaaggcttgaagaatccatctctctcaagctcagcacgccatctagcgaaatcctcaagcataggagcatcctcagactcagatctcttgatctcagcaggtctagaaggcaaagctctaagcatcttccaagccttgagagaacgcatgtggaattctttgaaagcctcagtagcatcagcaccagtgttagcaagcatgtagaagatcacagatccaccagggtgcttgaagttagtcacatcgtactcaacgtcctcaactctaacccatctagtctcgaaagtagcagcaagctcatgaggctcaagagtcttaagatcaacaggagcagtagaagcatccttagcatcaagagcctcagcagaagatttagacctggtaagtggagatctaggagaagatcttccatcagtcttaggagggcacatggtatggtaattgtaaatgtaattgtaatgttgtttgttgtttgttgttgttggtaattgttgtaaaattaattaagtgggtatcttttggatggataagcaagtagtgatgatgttctaggtgaagtgatgggggtgttttatagcgggagatggtgaaatggatggtcgccacataagaaatggaggggaagggttcttgcgccattcttcagtttgcatggatgcatgggtttcattttgtaacacgtaataaggacaatgaagtgcaggtgtctctcaagtttcagaggggatatgtggacagaagaagaacggcgatgatattgatggaaatggccatctagtgtgaatctattcggttgataatactagtgcattttggccgttaatcccttcaattaactgcacaaacttcagttgagtattgattatttgattataggttctgtaaacacaataccaagtttatttagaggggagacatacaaatagtttcgatataaataatagagtggttaaacttagttattaaaactatatataaagtctaaaagttaaattatttttttaattgcaaatatataaagtctaaaggggttacattatttcttaagagatgtaactctgttggaatctgacttaatccgtctcatcactctggtttccagttctaatctaatgaattgttttctgccaaagaatttgaagcaagaagtaaattgatcaatgccgtcaacccacaccaaaccgtcaacccactaccatcgccgcggagacccccaaactcaacctccacccatcggtaagaagcacagggcagcccgcaccaccaccaatttggcgtgcatgacacctagggacttggcacgggaggcggcgcacgtggatgcaaatgacgggatatcagatgacaggaaacgacgttgagagaccatacgatgtagaatatgagctcaccatcaacgagaaactaggaaaatcacaaaaaaaacaactctcgtaattgtacgagtggcacagatgggtctgcctcaacatatctctaatacggcgaagcctgcccaacacgtagttgccggaatccggtgtggagctcacgactctgaaagataggcgcttcctgtttcgtttcgctcacccactggacgtccgtcatgtgatggatttcggtcattggtttgctgacaaccacattctgaagctccatgagatgagtcttcacaataggtcctgctcaataccgtggagttatggttgcaagtccataacttgccgttcgaatattttgcggagccagtcggacgggaattggcgagctcggctgacacctataaaggccatgacaagaagaaccaaaagttcttccctaatgctttcatgaggcttcgggtcgttatggatgtcggaaaacccctcttgaaggaacgagacgttattatgcatgacggtaagactattacttgtcagtataagtatgaaagattacctgtcttctgctttgtttgtggattgattggacacgttgaaaaaaaatgtgcacttcgatttcaatactcagagatcgacttcccttttctctaggagtattcgatcaaggcattaacatggaaggaagctcaagctctaaaggcttcacaatggaacctgaaaaatttcaacaagcctaaactgaaatcgaagtcaaatcacccaaccgggagctctaaatcagcaaacactcctcctccacagtatccaatcatcgtgcacgatgctccaggtattgcaagccaggtattgcaagctaggagtaggatagagaccttaaacgtcgttggtgtgaagagtcatcttcagacctaatggagatagatgtagacggcggcacgaagactctgaaacaccagaaaggctagtccaggataaggatctgctatcccaactgacctctcgttagtcccaaggcctctcaactagagcaggaggaaggatggtcacaagactaggataatgatgtttccaatatgaacctgaatgtccatagctaatttttttagtcttgcttctgcactttttgtttattatgttctggtgactatgttatttacccttgtccgtatgcttgagggtaccctagtagattggttggttggtttccatgtaccagaaggcttaccctattagttgaaagttgaaactttgttccctactcaattcctagttgtgtaaatgtatgtatatgtaatgtgtataaaacgtagtacttaaatgactaggagtggttcttgagaccgatgagagatgggagcagaactaaagatgatgacataattaagaacgaatttgaaaggctcttaggtttgaatcctattcgagaatgtttttgtcaaagatagtggcgattttgaaccaaagaaaacatttaaaaaatcagtatccggttacgttcatgcaaatagaaagtggtctaggatctgattgtaattttagacttaaagagtctcttaagattcaatcctggctgtgtacaaaactacaaataatatattttagactatttggccttaactaaacttccactcattatttactgaggttagagaatagacttgcgaataaacacattcccgagaaatactcatgatcccataattagtcagagggtatgccaatcagatctaagaacacacattccctcaaattttaatgcacatgtaatcatagtttagcacaattcaaaaataatgtagtattaaagacagaaatttgtagacttttttttggcgttaaaagaagactaagtttatacgtacattttattttaagtggaaaaccgaaattttccatcgaaatatatgaatttagtatatatatttctgcaatgtactattttgctattttggcaactttcagtggactactactttattacaatgtgtatggatgcatgagtttgagtatacacatgtctaaatgcatgctttgtaaaacgtaacggaccacaaaagaggatccatacaaatacatctcatagcttcctccattattttccgacacaaacagagcattttacaacaattaccaacaacaacaaacaacaaacaacattacaattacatttacaattaccataccatggcctctatcgctatccctgctgctcttgctggaactcttggatacgttacctacaatgtggctaaccctgatatcccagcttctgagaaagttcctgcttacttcatgcaggttgagtactggggacctactatcggaactattggatacctcctcttcatctacttcggaaagcgtatcatgcagaacagatctcaacctttcggactcaagaacgctatgctcgtttacaacttctaccagaccttcttcaacagctactgcatctaccttttcgttacttctcatagggctcagggacttaaggtttggggaaacatccctgatatgactgctaactcttggggaatctctcaggttatctggcttcactacaacaacaagtacgttgagcttctcgacaccttcttcatggtgatgaggaagaagttcgaccagctttctttccttcacatctaccaccacactcttctcatctggtcatggttcgttgttatgaagcttgagcctgttggagattgctacttcggatcttctgttaacaccttcgtgcacgtgatcatgtactcttactacggacttgctgctcttggagttaactgtttctggaagaagtacatcacccagatccagatgcttcagttctgtatctgtgcttctcactctatctacaccgcttacgttcagaataccgctttctggcttccttaccttcaactctgggttatggtgaacatgttcgttctcttcgccaacttctaccgtaagaggtacaagtctaagggtgctaagaagcagtgataaggcgcgcggcgcgccgggccgccgccatgtgacagatcgaaggaagaaagtgtaataagacgactctcactactcgatcgctagtgattgtcattgttatatataataatgttatctttcacaacttatcgtaatgcatgtgaaactataacacattaatcctacttgtcatatgataacactctccccatttaaaactcttgtcaatttaaagatataagattctttaaatgattaaaaaaaatatattataaattcaatcactcctactaataaattattaattattatttattgattaaaaaaatacttatactaatttagtctgaatagaataattagattctagtctcatccccttttaaaccaacttagtaaacgtttttttttttaattttatgaagttaagtttttaccttgtttttaaaaagaatcgttcataagatgccatgccagaacattagctacacgttacacatagcatgcagccgcggagaattgtttttcttcgccacttgtcactcccttcaaacacctaagagcttctctctcacagcacacacatacaatcacatgcgtgcatgcattattacacgtgatcgccatgcaaatctcctttatagcctataaattaactcatccgcttcactctttactcaaaccaaaactcatcgatacaaacaagattaaaaacatacacgaggatcttttacaacaattaccaacaacaacaaacaacaaacaacattacaattacatttacaattaccataccatgcctccaagggactcttactcttatgctgctcctccttctgctcaacttcacgaagttgatactcctcaagagcacgacaagaaagagcttgttatcggagatagggcttacgatgttaccaacttcgttaagagacaccctggtggaaagatcattgcttaccaagttggaactgatgctaccgatgcttacaagcagttccatgttagatctgctaaggctgacaagatgcttaagtctcttccttctcgtcctgttcacaagggatactctccaagaagggctgatcttatcgctgatttccaagagttcaccaagcaacttgaggctgagggaatgttcgagccttctcttcctcatgttgcttacagacttgctgaggttatcgctatgcatgttgctggtgctgctcttatctggcatggatacactttcgctggaatcgctatgcttggagttgttcagggaagatgtggatggcttatgcatgagggtggacattactctctcactggaaacattgctttcgacagagctatccaagttgcttgttacggacttggatgtggaatgtctggtgcttggtggcgtaaccagcataacaagcaccatgctactcctcaaaagcttcagcacgatgttgatcttgatacccttcctctcgttgctttccatgagagaatcgctgctaaggttaagtctcctgctatgaaggcttggctttctatgcaagctaagcttttcgctcctgttaccactcttcttgttgctcttggatggcagctttaccttcatcctagacacatgctcaggactaagcactacgatgagcttgctatgctcggaatcagatacggacttgttggataccttgctgctaactacggtgctggatacgttctcgcttgttaccttctttacgttcagcttggagctatgtacatcttctgcaacttcgctgtttctcatactcacctccctgttgttgagcctaacgagcatgctacttgggttgagtacgctgctaaccacactactaactgttctccatcttggtggtgtgattggtggatgtcttaccttaactaccagatcgagcaccacctttacccttctatgcctcaattcagacaccctaagatcgctcctagagttaagcagcttttcgagaagcacggacttcactacgatgttagaggatacttcgaggctatggctgatactttcgctaaccttgataacgttgcccatgctcctgagaagaaaatgcagtaatgagatcgttcaaacatttggcaataaagtttcttaagattgaatcctgttgccggtcttgcgatgattatcatataatttctgttgaattacgttaagcacgtaataattaacatgtaatgcatgacgttatttatgagatgggtttttatgattagagtcccgcaattatacatttaatacgcgatagaaaacaaaatatagcgcgcaaactaggataaattatcgcgcgcggtgtcatctatgttactagatcggtcgattaaaaatcccaattatatttggtctaatttagtttggtattgagtaaaacaaattcgaaccaaaccaaaatataaatatatagtttttatatatatgcctttaagactttttatagaattttctttaaaaaatatctagaaatatttgcgactcttctggcatgtaatatttcgttaaatatgaagtgctccatttttattaactttaaataattggttgtacgatcactttcttatcaagtgttactaaaatgcgtcaatctctttgttcttccatattcatatgtcaaaatctatcaaaattcttatatatctttttcgaatttgaagtgaaatttcgataatttaaaattaaatagaacatatcattatttaggtatcatattgatttttatacttaattactaaatttggttaactttgaaagtgtacatcaacgaaaaattagtcaaacgactaaaataaataaatatcatgtgttattaagaaaattctcctataagaatattttaatagatcatatgtttgtaaaaaaaattaatttttactaacacatatatttacttatcaaaaatttgacaaagtaagattaaaataatattcatctaacaaaaaaaaaaccagaaaatgctgaaaacccggcaaaaccgaaccaatccaaaccgatatagttggtttggtttgattttgatataaaccgaaccaactcggtccatttgcacccctaatcataatagctttaatatttcaagatattattaagttaacgttgtcaatatcctggaaattttgcaaaatgaatcaagcctatatggctgtaatatgaatttaaaagcagctcgatgtggtggtaatatgtaatttacttgattctaaaaaaatatcccaagtattaataatttctgctaggaagaaggttagctacgatttacagcaaagccagaatacaaagaaccataaagtgattgaagctcgaaatatacgaaggaacaaatatttttaaaaaaatacgcaatgacttggaacaaaagaaagtgatatattttttgttcttaaacaagcatcccctctaaagaatggcagttttcctttgcatgtaactattatgctcccttcgttacaaaaattttggactactattgggaacttcttctgaaaatagtgatagaacccacacgagcatgtgctttccatttaattttaaaaaccaagaaacatacatacataacattccatcagcctctctctctttttattacggttaatgacttaaaacacatcttattatcccatccttaacacctagcagtgtctttatacgatctcatcgatcaccacttcaaaaccatgcagactgctgctgcccctggagctggcatcggctaggctgggtgccgcactgtcccggaaggtccctagcgacttgtttagattgatgggaccacctctcaacttcctgctgctgtccctgctgctggatgtcctgcctcatctggccgattgcacgctccagtcccctgcatgtgcactcgctcctcaattgcttaagatcatcgcagcagctatcgaagtgctggctctgttgccctcctccacggccttggttgtagtagtagctgccgccgcccttctggactttttcccacaggaaccgccgaataattcgatagaaccacacgagcatgtgctttcatttattttaaaaaccaagaaacatacataacatttcatcagcctctctctctctctctctctctctctctctctctctctctctctctctctctttattacagctgttacactaacttaaaacacattcatctcattattattattattatccatccttaacacctagcagtgtctttgtacgatctcataatcgatcaccccttcatcaggtatccttaggcttcactccaacgttgttgcagttacggaacatgtacacaccatcatggttctcaacgaactggcaagatctccaagttttccaaaggctaacccacatgttctcatcggtgtgtctgtagtgctctcccataactttcttgatgcactcggtagcttctctagcatggtagaatgggatccttgaaacgtagtgatggagcacatgagtctcgatgatgtcatggaagatgattccgaggattccgaactctctatcgatagtagcagcagcacccttagcgaaagtccactcttgagcatcgtaatgaggcatagaagaatcggtgtgctgaaggaaggtaacgaaaacaagccagtggttaacaaggatccaaggacagaaccatgtgatgaaagtaggccagaatccgaaaaccttgtaagcggtgtaaacagaagtgagggtagcaaggattccaagatcagaaagaacgatgtaccagtagtccttcttatcgaaaacagggctagaaggccagtagtgagacttgaagaacttagaaacaccagggtaaggttgtccagtagcgttagtagcaaggtaaagagaaagtcctccaagctgttggaacaagagagcgaaaacagagtagataggagtttcctcagcgatatcgtgaaggctggtaacttggtgcttctctttgaattcctcggcggtgtaaggaacgaaaaccatatctctggtcatgtgtccagtagccttatggtgcttagcatgagagaacttccagctgaagtaaggaaccataacaagagagtggagaacccatccaacggtatcgttaacccatccgtagttagagaaagcagaatgtccacactcatgtccaaggatccagattccgaatccgaaacaagagatagagaacacgtaagcagaccaagcagcgaatctaaggaattcgttagggagaagagggatgtaggtaagtccaacgtaagcgatagcagagatagccacgatatctctcaccacgtaagacatagacttcacgagagatctctcgtaacagtgcttagggatagcgtcaaggatatccttgatggtgtaatctggcaccttgaaaacgtttccgaaggtatcgatagcggtcttttgctgcttgaaagatgcaacgtttccagaacgcctaacggtcttagtagatccctcaaggatctcagatccagacacggtaaccttagacatggtatggtaattgtaaatgtaattgtaatgttgtttgttgtttgttgttgttggtaattgttgtaaaatttttggtggtgattggttctttaaggtgtgagagtgagttgtgagttgtgtggtgggtttggtgagattggggatggtgggtttatatagtggagactgaggaatggggtcgtgagtgttaactttgcatgggctacacgtgggttcttttgggcttacacgtagtattattcatgcaaatgcagccaatacatatacggtattttaataatgtgtgggaatacaatatgccgagtattttactaattttggcaatgacaagtgtacatttggattatcttacttggcctctcttgctttaatttggattatttttattctcttaccttggccgttcatattcacatccctaaaggcaagacagaattgaatggtggccaaaaattaaaacgatggatatgacctacatagtgtaggatcaattaacgtcgaaggaaaatactgattctgcccgttcgactcagatcttccaaggcctcgtctccgagtccgctgcttctcgccgcgccgatcacttctccgccgccaacaaggcttgtagttaataggaatcattcagggattgtgattccgggcagtagtaattaataatatagtattagtatacagaacctcttatttagctaaaagattatgttcttaatgttgataagaagtttgagaaacaaatataattgagcttctgattagttgatcgtaattggtcattaataattgtatctaaccagtgcagtataagagcgtataagagcatcttcaaaaagactttattttagagttaatcagtgcagtataagagcatctctaaaaaaactctaattatagagttttgcaaactctatatttgaagttttaaggtgtttttttttcaaaagcaaaacttcaaatttaacttcaaaattatttgtaatttacactatgctctttatatttatcataattaatataagggggtgttagtgggacttagatttctatagagtttgttgattttaaaagttgagagatttgttaaatttagaaagagatgtagagaattttgtctattgtgaaaatctatgaaaatagagtaatgtaatgattctaagaattcaaagtaaacatgtagtattctcaaaatctaaatttgtgaaacagtggtcccagattttcaagactcagactaaaggctatggaggaagctagggttttggcgattggcgacactagggtttcgagtacggcagatttggatgaaactatgatggatgtgggggagagagggagaccgccaggagatccgccagataagttaacctcatgggtagcgaaggtggtggagacggctgagggagggatgccagtaccggaggttttgattgcagattcttttgtgtcggagagggtacgggtagaatttccgaatg

SEQ ID NO: 41 - DNA, 49789 bp, synthetic construct
  misc_feature 1..49789: note = Chimeric 16 transgene inserted into Brassica
  source 1..49789: mol_type = other DNA
aaaaaatacaaccaaagaaaaatataccagaaggttgtgatttggtccattatataaaaattacgaaatgaatttctttatccttttatctcaaattttattgaagacttttgtaggattatagttgactttatgctcacatatatatacactgatcaaaactttttaaaaacataaagaaattgtgaaacaataaaaataaaatgaaatgagtaattaatgagtagattaagacattggaccctccacaggcgataaagtaaaataatcagaagttgcaggaggcaaaggaggactactactaatacttggaacttggaagtagctatcgtgcgcatctgcctccaagtccaacaccttataacaaatttccgccgggaagaaagaaaagtctctctgccctctcttctttagcctccagcttctgcaaaccatacgtacaaacaagatagacacaatcctccctacctccttcttctatcttcatcgaaagattcaaccaccactcaagtcttctctctcttttttggaaagaaaaaaggtaaaagctttcttctttctgagcaaactcccatgaatttcccttttgggggtttagggtctttccttttatgttcctacttcggtataattcgatttcatgcgaacttagattataaaaatttgatcttttttttgtggggtttgaaattgaaatccattttaggggttaccatcgttgaccaaatgtctcgactttgttcgaatcatgatgttacttaatcatggaggagaagaaggatttttataaccatgtctctgttgcttgctgcttaaaccctatataattggaaactttttgttttagtctgtgtctgaaagtttctatattcgtattgtctattttgtaaagactaaaacaaaaatgcctatttttagtttgttcttgttccgcaacaccgttactgaactcttcgttcacttaaacagtttgtgtgtgtgagaaacagcgtaatgagctgctttggttgttgtggtggtgacgattttcgtcgagttgctgaaactggacccaagccagtgtacggcgcaggaggtactttaagcttataaccctttgtctatcctttggctagcggctaatgttgatgaacttttttattcaaccgttggctaaggtaacactgatagtttaaactgaaggcgggaaacgacaatctgctagtggatctcccagtcacgacgttgtaaaacgggcgccccgcggaaagcttgcggccgcggtaccgcccgttcgactcagatcttccaaggcctcgtctccgagtccgctgcttctcgccgcgccgatcacttctccgccgccaacaaggcttgtagttaataggaatcattcagggattgtgattccgggcagtagtaattaataatatagtattagtatagataatatgtttcgtttgggatctttggaacgttgctctgttccttgttgttcattttaaagcttttgagggatagttgcagaactgttcggtgatgcttcatcctctcaagaactagatttgggtaaagaaacatccatgcatggatatggaatgttgttcttccgattggagattattttataaaatttaaaattcatgatttaaaaaaacacataaaaaccacaaaattcatgatttattgacaatacgatacaaaattagcaccaccggctactggctcattacacatttccccttcccctcattctcactttgtggctttattattattattattacatatattttaccgttattatttcacgtcacataagcttgttaattaatcattagtgagccttctcagcctttccgttaacgtagtagtgctgtcccaccttatcaaggttagagaaagtagccttccaagcaccgtagtaagagagcaccttgtagttgagtccccacttcttagcgaaaggaacgaatcttctgctaacctcaggctgtctgaattgaggcatatcagggaagaggtggtggataacctgacagttaaggtatcccataagccagttcacgtatcctctagaaggatcgatatcaacggtgtgatcaacagcgtagttaacccaagaaaggtgcttatcagatggaacaacagggaggtgagtatgagaagtagagaagtgagcgaaaaggtacatgtaagcgatccagtttccgaaagtgaaccaccagtaagcaacaggccaagagtatccagtagcaagcttgataacagcggttctaacaacatgagaaacgagcatccaagaagcctcttcgtagttcttcttacggagaacttgtctagggtggagaacgtagatccagaaagcttgaacaagaagtccagaggtaacaggaacgaaagtccaagcttgaagtctagcccaagctctagagaatcctctaggtctgttatcctcaacagcagtgttgaagaaagccacagcaggagtggtatcaagatccatatcgtgtctaaccttttgaggggtagcatggtgcttgttatgcatctggttccacatctcaccagaagtagaaagtccgaatccacaagtcatagcctgaagtctcttgtccacgtaaacagatccggtaagagagttatgtccaccctcatgttgaacccatccacatctagctccgaagaaagcaccgtaaacaacagaagcaatgatagggtatccagcgtacataagagcagttccaagagcgaatgtagcaagaagctcgagaagtctgtaagccacatgggtgatagaaggcttgaagaatccatctctctcaagctcagcacgccatctagcgaaatcctcaagcataggagcatcctcagactcagatctcttgatctcagcaggtctagaaggcaaagctctaagcatcttccaagccttgagagaacgcatgtggaattctttgaaagcctcagtagcatcagcaccagtgttagcaagcatgtagaagatcacagatccaccagggtgcttgaagttagtcacatcgtactcaacgtcctcaactctaacccatctagtctcgaaagtagcagcaagctcatgaggctcaagagtcttaagatcaacaggagcagtagaagcatccttagcatcaagagcctcagcagaagatttagacctggtaagtggagatctaggagaagatcttccatcagtcttaggagggcacatggtatggtaattgtaaatgtaattgtaatgttgtttgttgtttgttgttgttggtaattgttgtaaaattaattaagtgggtatcttttggatggataagcaagtagtgatgatgttctaggtgaagtgatgggggtgttttatagcgggagatggtgaaatggatggtcgccacataagaaatggaggggaagggttcttgcgccattcttcagtttgcatggatgcatgggtttcattttgtaacacgtaataaggacaatgaagtgcaggtgtctctcaagtttcagaggggatatgtggacagaagaagaacggcgatgatattgatggaaatggccatctagtgtgaatctattcggttgataatactagtgcattttggccgttaatcccttcaattaactgcacaaacttcagttgagtattgattatttgattataggttctgtaaacacaataccaagtttatttagaggggagacatacaaatagtttcgatataaataatagagtggttaaacttagttattaaaactatatataaagtctaaaagttaaattatttttttaattgcaaatatataaagtctaaaggggttacattatttcttaagagatgtaactctgttggaatctgacttaatccgtctcatcactctggtttccagttctaatctaatgaattgttttctgccaaagaatttgaagcaagaagtaaattgatcaatgccgtcaacccacaccaaaccgtcaacccactaccatcgccgcggagacccccaaactcaacctccacccatcggtaagaagcacagggcagcccgcaccaccaccaatttggcgtgcatgacacctagggacttggcacgggaggcggcgcacgtggatgcaaatgacgggatatcagatgacaggaaacgacgttgagagaccatacgatgtagaatatgagctcaccatcaacgagaaactaggaaaatcacaaaaaaaacaactctcgtaattgtacgagtggcacagatgggtctgcctcaacatatctctaatacggcgaagcctgcccaacacgtagttgccggaatccggtgtggagctcacgactctgaaagataggcgcttcctgtttcgtttcgctcacccactggacgtccgtcatgtgatggatttcggtcattggtttgctgacaaccacattctgaagctccatgagatgagtcttcacaataggtcctgctcaataccgtggagttatggttgcaagtccataacttgccgttcgaatattttgcggagccagtcggacgggaattggcgagctcggctgacacctataaaggccatgacaagaagaaccaaaagttcttccctaatgctttcatgaggcttcgggtcgttatggatgtcggaaaacccctcttgaaggaacgagacgttattatgcatgacggtaagactattacttgtcagtataagtatgaaagattacctgtcttctgctttgtttgtggattgattggacacgttgaaaaaaaatgtgcacttcgatttcaatactcagagatcgacttcccttttctctaggagtattcgatcaaggcattaacatggaaggaagctcaagctctaaaggcttcacaatggaacctgaaaaatttcaacaagcctaaactgaaatcgaagtcaaatcacccaaccgggagctctaaatcagcaaacactcctcctccacagtatccaatcatcgtgcacgatgctccaggtattgcaagccaggtattgcaagctaggagtaggatagagaccttaaacgtcgttggtgtgaagagtcatcttcagacctaatggagatagatgtagacggcggcacgaagactctgaaacaccagaaaggctagtccaggataaggatctgctatcccaactgacctctcgttagtcccaaggcctctcaactagagcaggaggaaggatggtcacaagactaggataatgatgtttccaatatgaacctgaatgtccatagctaatttttttagtcttgcttctgcactttttgtttattatgttctggtgactatgttatttacccttgtccgtatgcttgagggtaccctagtagattggttggttggtttccatgtaccagaaggcttaccctattagttgaaagttgaaactttgttccctactcaattcctagttgtgtaaatgtatgtatatgtaatgtgtataaaacgtagtacttaaatgactaggagtggttcttgagaccgatgagagatgggagcagaactaaagatgatgacataattaagaacgaatttgaaaggctcttaggtttgaatcctattcgagaatgtttttgtcaaagatagtggcgattttgaaccaaagaaaacatttaaaaaatcagtatccggttacgttcatgcaaatagaaagtggtctaggatctgattgtaattttagacttaaagagtctcttaagattcaatcctggctgtgtacaaaactacaaataatatattttagactatttggccttaactaaacttccactcattatttactgaggttagagaatagacttgcgaataaacacattcccgagaaatactcatgatcccataattagtcagagggtatgccaatcagatctaagaacacacattccctcaaattttaatgcacatgtaatcatagtttagcacaattcaaaaataatgtagtattaaagacagaaatttgtagacttttttttggcgttaaaagaagactaagtttatacgtacattttattttaagtggaaaaccgaaattttccatcgaaatatatgaatttagtatatatatttctgcaatgtactattttgctattttggcaactttcagtggactactactttattacaatgtgtatggatgcatgagtttgagtatacacatgtctaaatgcatgctttgtaaaacgtaacggaccacaaaagaggatccatacaaatacatctcatagcttcctccattattttccgacacaaacagagcattttacaacaattaccaacaacaacaaacaacaaacaacattacaattacatttacaattaccataccatggcctctatcgctatccctgctgctcttgctggaactcttggatacgttacctacaatgtggctaaccctgatatcccagcttctgagaaagttcctgcttacttcatgcaggttgagtactggggacctactatcggaactattggatacctcctcttcatctacttcggaaagcgtatcatgcagaacagatctcaacctttcggactcaagaacgctatgctcgtttacaacttctaccagaccttcttcaacagctactgcatctaccttttcgttacttctcatagggctcagggacttaaggtttggggaaacatccctgatatgactgctaactcttggggaatctctcaggttatctggcttcactacaacaacaagtacgttgagcttctcgacaccttcttcatggtgatgaggaagaagttcgaccagctttctttccttcacatctaccaccacactcttctcatctggtcatggttcgttgttatgaagcttgagcctgttggagattgctacttcggatcttctgttaacaccttcgtgcacgtgatcatgtactcttactacggacttgctgctcttggagttaactgtttctggaagaagtacatcacccagatccagatgcttcagttctgtatctgtgcttctcactctatctacaccgcttacgttcagaataccgctttctggcttccttaccttcaactctgggttatggtgaacatgttcgttctcttcgccaacttctaccgtaagaggtacaagtctaagggtgctaagaagcagtgataaggcgcgcggcgcgccgggccgccgccatgtgacagatcgaaggaagaaagtgtaataagacgactctcactactcgatcgctagtgattgtcattgttatatataataatgttatctttcacaacttatcgtaatgcatgtgaaactataacacattaatcctacttgtcatatgataacactctccccatttaaaactcttgtcaatttaaagatataagattctttaaatgattaaaaaaaatatattataaattcaatcactcctactaataaattattaattattatttattgattaaaaaaatacttatactaatttagtctgaatagaataattagattctagtctcatccccttttaaaccaacttagtaaacgtttttttttttaattttatgaagttaagtttttaccttgtttttaaaaagaatcgttcataagatgccatgccagaacattagctacacgttacacatagcatgcagccgcggagaattgtttttcttcgccacttgtcactcccttcaaacacctaagagcttctctctcacagcacacacatacaatcacatgcgtgcatgcattattacacgtgatcgccatgcaaatctcctttatagcctataaattaactcatccgcttcactctttactcaaaccaaaactcatcgatacaaacaagattaaaaacatacacgaggatcttttacaacaattaccaacaacaacaaacaacaaacaacattacaattacatttacaattaccataccatgcctccaagggactcttactcttatgctgctcctccttctgctcaacttcacgaagttgatactcctcaagagcacgacaagaaagagcttgttatcggagatagggcttacgatgttaccaacttcgttaagagacaccctggtggaaagatcattgcttaccaagttggaactgatgctaccgatgcttacaagcagttccatgttagatctgctaaggctgacaagatgcttaagtctcttccttctcgtcctgttcacaagggatactctccaagaagggctgatcttatcgctgatttccaagagttcaccaagcaacttgaggctgagggaatgttcgagccttctcttcctcatgttgcttacagacttgctgaggttatcgctatgcatgttgctggtgctgctcttatctggcatggatacactttcgctggaatcgctatgcttggagttgttcagggaagatgtggatggcttatgcatgagggtggacattactctctcactggaaacattgctttcgacagagctatccaagttgcttgttacggacttggatgtggaatgtctggtgcttggtggcgtaaccagcataacaagcaccatgctactcctcaaaagcttcagcacgatgttgatcttgatacccttcctctcgttgctttccatgagagaatcgctgctaaggttaagtctcctgctatgaaggcttggctttctatgcaagctaagcttttcgctcctgttaccactcttcttgttgctcttggatggcagctttaccttcatcctagacacatgctcaggactaagcactacgatgagcttgctatgctcggaatcagatacggacttgttggataccttgctgctaactacggtgctggatacgttctcgcttgttaccttctttacgttcagcttggagctatgtacatcttctgcaacttcgctgtttctcatactcacctccctgttgttgagcctaacgagcatgctacttgggttgagtacgctgctaaccacactactaactgttctccatcttggtggtgtgattggtggatgtcttaccttaactaccagatcgagcaccacctttacccttctatgcctcaattcagacaccctaagatcgctcctagagttaagcagcttttcgagaagcacggacttcactacgatgttagaggatacttcgaggctatggctgatactttcgctaaccttgataacgttgcccatgctcctgagaagaaaatgcagtaatgagatcgttcaaacatttggcaataaagtttcttaagattgaatcctgttgccggtcttgcgatgattatcatataatttctgttgaattacgttaagcacgtaataattaacatgtaatgcatgacgttatttatgagatgggtttttatgattagagtcccgcaattatacatttaatacgcgatagaaaacaaaatatagcgcgcaaactaggataaattatcgcgcgcggtgtcatctatgttactagatcggtcgattaaaaatcccaattatatttggtctaatttagtttggtattgagtaaaacaaattcgaaccaaaccaaaatataaatatatagtttttatatatatgcctttaagactttttatagaattttctttaaaaaatatctagaaatatttgcgactcttctggcatgtaatatttcgttaaatatgaagtgctccatttttattaactttaaataattggttgtacgatcactttcttatcaagtgttactaaaatgcgtcaatctctttgttcttccatattcatatgtcaaaatctatcaaaattcttatatatctttttcgaatttgaagtgaaatttcgataatttaaaattaaatagaacatatcattatttaggtatcatattgatttttatacttaattactaaatttggttaactttgaaagtgtacatcaacgaaaaattagtcaaacgactaaaataaataaatatcatgtgttattaagaaaattctcctataagaatattttaatagatcatatgtttgtaaaaaaaattaatttttactaacacatatatttacttatcaaaaatttgacaaagtaagattaaaataatattcatctaacaaaaaaaaaaccagaaaatgctgaaaacccggcaaaaccgaaccaatccaaaccgatatagttggtttggtttgattttgatataaaccgaaccaactcggtccatttgcacccctaatcataatagctttaatatttcaagatattattaagttaacgttgtcaatatcctggaaattttgcaaaatgaatcaagcctatatggctgtaatatgaatttaaaagcagctcgatgtggtggtaatatgtaatttacttgattctaaaaaaatatcccaagtattaataatttctgctaggaagaaggttagctacgatttacagcaaagccagaatacaaagaaccataaagtgattgaagctcgaaatatacgaaggaacaaatatttttaaaaaaatacgcaatgacttggaacaaaagaaagtgatatattttttgttcttaaacaagcatcccctctaaagaatggcagttttcctttgcatgtaactattatgctcccttcgttacaaaaattttggactactattgggaacttcttctgaaaatagtgatagaacccacacgagcatgtgctttccatttaattttaaaaaccaagaaacatacatacataacattccatcagcctctctctctttttattacggttaatgacttaaaacacatcttattatcccatccttaacacctagcagtgtctttatacgatctcatcgatcaccacttcaaaaccatgcagactgctgctgcccctggagctggcatcggctaggctgggtgccgcactgtcccggaaggtccctagcgacttgtttagattgatgggaccacctctcaacttcctgctgctgtccctgctgctggatgtcctgcctcatctggccgattgcacgctccagtcccctgcatgtgcactcgctcctcaattgcttaagatcatcgcagcagctatcgaagtgctggctctgttgccctcctccacggccttggttgtagtagtagctgccgccgcccttctggactttttcccacaggaaccgccgaataattcgatagaaccacacgagcatgtgctttcatttattttaaaaaccaagaaacatacataacatttcatcagcctctctctctctctctctctctctctctctctctctctctctctctctctctttattacagctgttacactaacttaaaacacattcatctcattattattattattatccatccttaacacctagcagtgtctttgtacgatctcataatcgatcaccccttcatcaggtatccttaggcttcactccaacgttgttgcagttacggaacatgtacacaccatcatggttctcaacgaactggcaagatctccaagttttccaaaggctaacccacatgttctcatcggtgtgtctgtagtgctctcccataactttcttgatgcactcggtagcttctctagcatggtagaatgggatccttgaaacgtagtgatggagcacatgagtctcgatgatgtcatggaagatgattccgaggattccgaactctctatcgatagtagcagcagcacccttagcgaaagtccactcttgagcatcgtaatgaggcatagaagaatcggtgtgctgaaggaaggtaacgaaaacaagccagtggttaacaaggatccaaggacagaaccatgtgatgaaagtaggccagaatccgaaaaccttgtaagcggtgtaaacagaagtgagggtagcaaggattccaagatcagaaagaacgatgtaccagtagtccttcttatcgaaaacagggctagaaggccagtagtgagacttgaagaacttagaaacaccagggtaaggttgtccagtagcgttagtagcaaggtaaagagaaagtcctccaagctgttggaacaagagagcgaaaacagagtagataggagtttcctcagcgatatcgtgaaggctggtaacttggtgcttctctttgaattcctcggcggtgtaaggaacgaaaaccatatctctggtcatgtgtccagtagccttatggtgcttagcatgagagaacttccagctgaagtaaggaaccataacaagagagtggagaacccatccaacggtatcgttaacccatccgtagttagagaaagcagaatgtccacactcatgtccaaggatccagattccgaatccgaaacaagagatagagaacacgtaagcagaccaagcagcgaatctaaggaattcgttagggagaagagggatgtaggtaagtccaacgtaagcgatagcagagatagccacgatatctctcaccacgtaagacatagacttcacgagagatctctcgtaacagtgcttagggatagcgtcaaggatatccttgatggtgtaatctggcaccttgaaaacgtttccgaaggtatcgatagcggtcttttgctgcttgaaagatgcaacgtttccagaacgcctaacggtcttagtagatccctcaaggatctcagatccagacacggtaaccttagacatggtatggtaattgtaaatgtaattgtaatgttgtttgttgtttgttgttgttggtaattgttgtaaaatttttggtggtgattggttctttaaggtgtgagagtgagttgtgagttgtgtggtgggtttggtgagattggggatggtgggtttatatagtggagactgaggaatggggtcgtgagtgttaactttgcatgggctacacgtgggttcttttgggcttacacgtagtattattcatgcaaatgcagccaatacatatacggtattttaataatgtgtgggaatacaatatgccgagtattttactaattttggcaatgacaagtgtacatttggattatcttacttggcctctcttgctttaatttggattatttttattctcttaccttggccgttcatattcacatccctaaaggcaagacagaattgaatggtggccaaaaattaaaacgatggatatgacctacatagtgtaggatcaattaacgtcgaaggaaaatactgattctctcaagcatacggacaagggtaaataacatagtcaccagaacataataaacaaaaagtgcagaagcaagactaaaaaaattagctatggacattcaggttcatattggaaacatcattatcctagtcttgtgaccatccttcctcctgctctagttgagaggccttgggactaacgagaggtcagttgggatagcagatccttatcctggactagcctttctggtgtttcagagtcttcgtgccgccgtctacatctatctccattaggtctgaagatgactcttcacaccaacgacgtttaaggtctctatcctactcctagcttgcaatacctggcttgcaatacctggagcatcgtgcacgatgattggatactgtggaggaggagtgtttgctgatttagagctcccggttgggtgatttgacttcgatttcagtttaggcttgttgaaatttttcaggttccattgtgaagcctttagagcttgagcttccttccatgttaatgccttgatcgaatactcctagagaaaagggaagtcgatctctgagtattgaaatcgaagtgcacattttttttcaacgtgtccaatcaatccacaaacaaagcagaagacaggtaatctttcatacttatactgacaagtaatagtcttaccgtcatgcataataacgtctcgttccttcaagaggggttttccgacatccataacgacccgaagcctcatgaaagcattagggaagaacttttggttcttcttgtcatggcctttataggtgtcagccgagctcgccaattcccgtccgactggctccgcaaaatattcgaacggcaagttatggacttgcaaccataactccacggtattgagcaggacctattgtgaagactcatctcatggagcttcagaatgtggttgtcagcaaaccaatgaccgaaatccatcacatgacggacgtccagtgggtgagcgaaacgaaacaggaagcgcctatctttcagagtcgtgagctccacaccggattccggcaactacgtgttgggcaggcttcgccgtattagagatatgttgaggcagacccatctgtgccactcgtacaattacgagagttgttttttttgtgattttcctagtttctcgttgatggtgagctcatattctacatcgtatggtctctcaacgtcgtttcctgtcatctgatatcccgtcatttgcatccacgtgcgccgcctcccgtgccaagtccctaggtgtcatgcacgccaaattggtggtggtgcgggctgccctgtgcttcttaccgatgggtggaggttgagtttgggggtctccgcggcgatggtagtgggttgacggtttggtgtgggttgacggcattgatcaatttacttcttgcttcaaattctttggcagaaaacaattcattagattagaactggaaaccagagtgatgagacggattaagtcagattccaacagagttacatctcttaagaaataatgtaacccctttagactttatatatttgcaattaaaaaaataatttaacttttagactttatatatagttttaataactaagtttaaccactctattatttatatcgaaactatttgtatgtctcccctctaaataaacttggtattgtgtttacagaacctataatcaaataatcaatactcaactgaagtttgtgcagttaattgaagggattaacggccaaaatgcactagtattatcaaccgaatagattcacactagatggccatttccatcaatatcatcgccgttcttcttctgtccacatatcccctctgaaacttgagagacacctgcacttcattgtccttattacgtgttacaaaatgaaacccatgcatccatgcaaactgaagaatggcgcaagaacccttcccctccatttcttatgtggcgaccatccatttcaccatctcccgctataaaacacccccatcacttcacctagaacatcatcactacttgcttatccatccaaaagatacccacttttacaacaattaccaacaacaacaaacaacaaacaacattacaattacatttacaattaccataccatgccacctagcgctgctaagcaaatgggagcttctactggtgttcatgctggtgttactgactcttctgctttcaccagaaaggatgttgctgatagacctgatctcaccatcgttggagattctgtttacgatgctaaggctttcagatctgagcatcctggtggtgctcatttcgtttctttgttcggaggaagagatgctactgaggctttcatggaataccatagaagggcttggcctaagtctagaatgtctagattccacgttggatctcttgcttctactgaggaacctgttgctgctgatgagggataccttcaactttgtgctaggatcgctaagatggtgccttctgtttcttctggattcgctcctgcttcttactgggttaaggctggacttatccttggatctgctatcgctcttgaggcttacatgctttacgctggaaagagacttctcccttctatcgttcttggatggcttttcgctcttatcggtcttaacatccagcatgatgctaaccatggtgctttgtctaagtctgcttctgttaaccttgctcttggactttgtcaggattggatcggaggatctatgatcctttggcttcaagagcatgttgttatgcaccacctccacactaacgatgttgataaggatcctgatcaaaaggctcacggtgctcttagactcaagcctactgatgcttggtcacctatgcattggcttcagcatctttaccttttgcctggtgagactatgtacgctttcaagcttttgttcctcgacatctctgagcttgttatgtggcgttgggagggtgagcctatctctaagcttgctggatacctctttatgccttctttgcttctcaagcttaccttctgggctagattcgttgctttgcctctttaccttgctccttctgttcatactgctgtgtgtatcgctgctactgttatgactggatctttctacctcgctttcttcttcttcatctcccacaacttcgagggtgttgcttctgttggacctgatggatctatcacttctatgactagaggtgctagcttccttaagagacaagctgagacttcttctaacgttggaggacctcttcttgctactcttaacggtggactcaactaccaaattgagcatcacttgttccctagagttcaccatggattctaccctagacttgctcctcttgttaaggctgagcttgaggctagaggaatcgagtacaagcactaccctactatctggtctaaccttgcttctaccctcagacatatgtacgctcttggaagaaggcctagatctaaggctgagtaatgacaagcttatgtgacgtgaaataataacggtaaaatatatgtaataataataataataaagccacaaagtgagaatgaggggaaggggaaatgtgtaatgagccagtagccggtggtgctaattttgtatcgtattgtcaataaatcatgaattttgtggtttttatgtgtttttttaaatcatgaattttaaattttataaaataatctccaatcggaagaacaacattccatatccatgcatggatgtttctttacccaaatctagttcttgagaggatgaagcatcaccgaacagttctgcaactatccctcaaaagctttaaaatgaacaacaaggaacagagcaacgttccaaagatcccaaacgaaacatattatctatactaatactatattattaattactactgcccggaatcacaatccctgaatgattcctattaactacaagccttgttggcggcggagaagtgatcggcgcggcgagaagcagcggactcggagacgaggccttggaagatctgagtcgaacgggcagaatcagtattttccttcgacgttaattgatcctacactatgtaggtcatatccatcgttttaatttttggccaccattcaattctgtcttgcctttagggatgtgaatatgaacggccaaggtaagagaataaaaataatccaaattaaagcaagagaggccaagtaagataatccaaatgtacacttgtcattgccaaaattagtaaaatactcggcatattgtattcccacacattattaaaataccgtatatgtattggctgcatttgcatgaataatactacgtgtaagcccaaaagaacccacgtgtagcccatgcaaagttaacactcacgaccccattcctcagtctccactatataaacccaccatccccaatctcaccaaacccaccacacaactcacaactcactctcacaccttaaagaaccaatcaccaccaaaaattttacaacaattaccaacaacaacaaacaacaaacaacattacaattacatttacaattaccataccatgagcgctgttaccgttactggatctgatcctaagaacagaggatcttctagcaacaccgagcaagaggttccaaaagttgctatcgataccaacggaaacgtgttctctgttcctgatttcaccatcaaggacatccttggagctatccctcatgagtgttacgagagaagattggctacctctctctactacgtgttcagagatatcttctgcatgcttaccaccggataccttacccataagatcctttaccctctcctcatctcttacacctctaacagcatcatcaagttcactttctgggccctttacacttacgttcaaggacttttcggaaccggaatctgggttctcgctcatgagtgtggacatcaagctttctctgattacggaatcgtgaacgatttcgttggatggacccttcactcttaccttatggttccttacttcagctggaagtactctcatggaaagcaccataaggctactggacacatgaccagagatatggttttcgttcctgccaccaaagaggaattcaagaagtctaggaacttcttcggtaacctcgctgagtactctgaggattctccacttagaaccctttacgagcttcttgttcaacaacttggaggatggatcgcttacctcttcgttaacgttacaggacaaccttaccctgatgttccttcttggaaatggaaccacttctggcttacctctccacttttcgagcaaagagatgctctctacatcttcctttctgatcttggaatcctcacccagggaatcgttcttactctttggtacaagaaattcggaggatggtcccttttcatcaactggttcgttccttacatctgggttaaccactggctcgttttcatcacattccttcagcacactgatcctactatgcctcattacaacgctgaggaatggactttcgctaagggtgctgctgctactatcgatagaaagttcggattcatcggacctcacatcttccatgatatcatcgagactcatgtgcttcaccactactgttctaggatcccattctacaacgctagacctgcttctgaggctatcaagaaagttatgggaaagcactacaggtctagcgacgagaacatgtggaagtcactttggaagtctttcaggtcttgccaatacgttgacggtgataacggtgttctcatgttccgtaacatcaacaactgcggagttggagctgctgagaagtaatgaaggggtgatcgattatgagatcgtacaaagacactgctaggtgttaaggatggataataataataataatgagatgaatgtgttttaagttagtgtaacagctgtaataaagagagagagagagagagagagagagagagagagagagagagagagagagaggctgatgaaatgttatgtatgtttcttggtttttaaaataaatgaaagcacatgctcgtgtggttctatcgaattattcggcggttcctgtgggaaaaagtccagaagggccgccgcagctactactacaaccaaggccgtggaggagggcaacagagccagcacttcgatagctgctgcgatgatcttaagcaattgaggagcgagtgcacatgcaggggactggagcgtgcaatcggccagatgaggcaggacatccagcagcagggacagcagcaggaagttgagaggtggtcccatcaatctaaacaagtcgctagggaccttccgggacagtgcggcacccagcctagccgatgccagctccaggggcagcagcagtctgcatggttttgaagtggtgatcgatgagatcgtataaagacactgctaggtgttaaggatgggataataagatgtgttttaagtcattaaccgtaataaaaagagagagaggctgatggaatgttatgtatgtatgtttcttggtttttaaaattaaatggaaagcacatgctcgtgtgggttctatctcgattaaaaatcccaattatatttggtctaatttagtttggtattgagtaaaacaaattcgaaccaaaccaaaatataaatatatagtttttatatatatgcctttaagactttttatagaattttctttaaaaaatatctagaaatatttgcgactcttctggcatgtaatatttcgttaaatatgaagtgctccatttttattaactttaaataattggttgtacgatcactttcttatcaagtgttactaaaatgcgtcaatctctttgttcttccatattcatatgtcaaaatctatcaaaattcttatatatctttttcgaatttgaagtgaaatttcgataatttaaaattaaatagaacatatcattatttaggtatcatattgatttttatacttaattactaaatttggttaactttgaaagtgtacatcaacgaaaaattagtcaaacgactaaaataaataaatatcatgtgttattaagaaaattctcctataagaatattttaatagatcatatgtttgtaaaaaaaattaatttttactaacacatatatttacttatcaaaaatttgacaaagtaagattaaaataatattcatctaacaaaaaaaaaaccagaaaatgctgaaaacccggcaaaaccgaaccaatccaaaccgatatagttggtttggtttgattttgatataaaccgaaccaactcggtccatttgcacccctaatcataatagctttaatatttcaagatattattaagttaacgttgtcaatatcctggaaattttgcaaaatgaatcaagcctatatggctgtaatatgaatttaaaagcagctcgatgtggtggtaatatgtaatttacttgattctaaaaaaatatcccaagtattaataatttctgctaggaagaaggttagctacgatttacagcaaagccagaatacaaagaaccataaagtgattgaagctcgaaatatacgaaggaacaaatatttttaaaaaaatacgcaatgacttggaacaaaagaaagtgatatattttttgttcttaaacaagcatcccctctaaagaatggcagttttcctttgcatgtaactattatgctcccttcgttacaaaaattttggactactattgggaacttcttctgaaaatagtcctgcaggctagtagattggttggttggtttccatgtaccagaaggcttaccctattagttgaaagttgaaactttgttccctactcaattcctagttgtgtaaatgtatgtatatgtaatgtgtataaaacgtagtacttaaatgactaggagtggttcttgagaccgatgagagatgggagcagaactaaagatgatgacataattaagaacgaatttgaaaggctcttaggtttgaatcctattcgagaatgtttttgtcaaagatagtggcgattttgaaccaaagaaaacatttaaaaaatcagtatccggttacgttcatgcaaatagaaagtggtctaggatctgattgtaattttagacttaaagagtctcttaagattcaatcctggctgtgtacaaaactacaaataatatattttagactatttggccttaactaaacttccactcattatttactgaggttagagaatagacttgcgaataaacacattcccgagaaatactcatgatcccataattagtcagagggtatgccaatcagatctaagaacacacattccctcaaattttaatgcacatgtaatcatagtttagcacaattcaaaaataatgtagtattaaagacagaaatttgtagacttttttttggcgttaaaagaagactaagtttatacgtacattttattttaagtggaaaaccgaaattttccatcgaaatatatgaatttagtatatatatttctgcaatgtactattttgctattttggcaactttcagtggactactactttattacaatgtgtatggatgcatgagtttgagtatacacatgtctaaatgcatgctttgtaaaacgtaacggaccacaaaagaggatccatacaaatacatctcatagcttcctccattattttccgacacaaacagagcattttacaacaattaccaacaacaacaaacaacaaacaacattacaattacatttacaattaccataccatggaatttgctcaacctctcgttgctatggctcaagagcagtacgctgctatcgatgctgttgttgctcctgctatcttctctgctaccgactctattggatggggactcaagcctatctcttctgctactaaggatctccctctcgttgaatctcctacccctcttatcctttctctcctcgcttacttcgctatcgttggttctggactcgtttaccgtaaagtgttccctagaaccgttaagggacaggatcctttccttctcaaggctcttatgctcgctcacaacgttttccttatcggactcagcctttacatgtgcctcaagctcgtttacgaggcttacgtgaacaagtactccttctggggaaacgcttacaaccctgctcaaaccgagatggctaaggtgatctggatcttctacgtgtccaagatctacgagttcatggacaccttcatcatgcttctcaagggaaacgttaaccaggtttccttcctccatgtttaccaccacggatctatctctggaatctggtggatgatcacttatgctgctccaggtggagatgcttacttctctgctgctctcaactcttgggttcatgtgtgcatgtacacctactacttcatggctgctgttcttcctaaggacgaaaagaccaagagaaagtacctttggtggggaagataccttacccagatgcaaatgttccagttcttcatgaaccttctccaggctgtttacctcctctactcttcttctccttaccctaagttcattgctcaactcctcgttgtttacatggttaccctcctcatgcttttcggaaacttctactacatgaagcaccacgcttctaagtgataagggccgccgccatgtgacagatcgaaggaagaaagtgtaataagacgactctcactactcgatcgctagtgattgtcattgttatatataataatgttatctttcacaacttatcgtaatgcatgtgaaactataacacattaatcctacttgtcatatgataacactctccccatttaaaactcttgtcaatttaaagatataagattctttaaatgattaaaaaaaatatattataaattcaatcactcctactaataaattattaattattatttattgattaaaaaaatacttatactaatttagtctgaatagaataattagattctagcctgcagggcggccgcggatcccatggagtcaaagattcaaatagaggacctaacagaactcgccgtaaagactggcgaacagttcatacagagtctcttacgactcaatgacaagaagaaaatcttcgtcaacatggtggagcacgacacacttgtctactccaaaaatatcaaagatacagtctcagaagaccaaagggcaattgagacttttcaacaaagggtaatatccggaaacctcctcggattccattgcccagctatctgtcactttattgtgaagatagtggaaaaggaaggtggctcctacaaatgccatcattgcgataaaggaaaggccatcgttgaagatgcctctgccgacagtggtcccaaagatggacccccacccacgaggagcatcgtggaaaaagaagacgttccaaccacgtcttcaaagcaagtggattgatgtgatatctccactgacgtaagggatgacgcacaatcccactatccttcgcaagacccttcctctatataaggaagttcatttcatttggagagaacacgggggactgaattaaatatgagccctgagaggcgtcctgttgaaatcagacctgctactgctgctgatatggctgctgtttgtgatatcgtgaaccactacatcgagacttctaccgttaacttcagaactgagcctcaaactcctcaagagtggatcgatgatcttgagagactccaagatagatacccttggcttgttgctgaggttgagggtgttgttgctggaatcgcttacgctggaccttggaaggctagaaacgcttacgattggactgttgagtctaccgtttacgtttcacacagacatcagagacttggacttggatctaccctttacactcaccttctcaagtctatggaagctcagggattcaagtctgttgttgctgttatcggactccctaacgatccttctgttagacttcatgaggctcttggatacactgctagaggaactcttagagctgctggatacaagcacggtggatggcatgatgttggattctggcaaagagatttcgagcttcctgctcctcctagacctgttagaccagttactcagatctgaatttgcgtgatcgttcaaacatttggcaataaagtttcttaagattgaatcctgttgccggtcttgcgatgattatcatataatttctgttgaattacgttaagcatgtaataattaacatgtaatgcatgacgttatttatgagatgggtttttatgattagagtcccgcaattatacatttaatacgcgatagaaaacaaaatatagcgcgcaaactaggataaattatcgcgcgcggtgtcatctatgttactagatcactagtgatgtacggttaaaaccaccccagtacattaaaaacgtccgcaatgtgttattaagttgtctaagcgtcaatttgtttacaccacaatatattgtggtgtaaacaaattgacgcttagacaacttaataacacattgcggacgtttttaatgtactggggtggttttaaccgtacatcactagtgatctagtaacatagatgacaccgcgcgcgataatttatcctagtttgcgcgctatattttgttttctatcgcgtattaaatgtataattgcgggactctaatcataaaaacccatctcataaataacgtcatgcattacatgttaattattacatgcttaacgtaattcaacagaaattatatgataatcatcgcaagaccggcaacaggattcaatcttaagaaactttattgccaaatgtttgaacgatcacgcaaattcagatctgagtaactggtctaacaggtctaggaggagcaggaagctcgaaatctctttgccagaatccaacatcatgccatccaccgtgcttgtatccagcagctctaagagttcctctagcagtgtatccaagagcctcatgaagtctaacagaaggatcgttagggagtccgataacagcaacaacagacttgaatccctgagcttccatagacttgagaaggtgagtgtaaagggtagatccaagtccaagtctctgatgtctgtgtgaaacgtaaacggtagactcaacagtccaatcgtaagcgtttctagccttccaaggtccagcgtaagcgattccagcaacaacaccctcaacctcagcaacaagccaagggtatctatcttggagtctctcaagatcatcgatccactcttgaggagtttgaggctcagttctgaagttaacggtagaagtctcgatgtagtggttcacgatatcacaaacagcagccatatcagcagcagtagcaggtctgatttcaacaggacgcctctcagggctcatatttaattcagtcccccgtgttctctccaaatgaaatgaacttccttatatagaggaagggtcttgcgaaggatagtgggattgtgcgtcatcccttacgtcagtggagatatcacatcaatccacttgctttgaagacgtggttggaacgtcttctttttccacgatgctcctcgtgggtgggggtccatctttgggaccactgtcggcagaggcatcttcaacgatggcctttcctttatcgcaatgatggcatttgtaggagccaccttccttttccactatcttcacaataaagtgacagatagctgggcaatggaatccgaggaggtttccggatattaccctttgttgaaaagtctcaattgccctttggtcttctgagactgtatctttgatatttttggagtagacaagtgtgtcgtgctccaccatgttgacgaagattttcttcttgtcattgagtcgtaagagactctgtatgaactgttcgccagtctttacggcgagttctgttaggtcctctatttgaatctttgactccatgggatccgcggccgccctgcaggctagaatctaattattctattcagactaaattagtataagtatttttttaatcaataaataataattaataatttattagtaggagtgattgaatttataatatattttttttaatcatttaaagaatcttatatctttaaattgacaagagttttaaatggggagagtgttatcatatgacaagtaggattaatgtgttatagtttcacatgcattacgataagttgtgaaagataacattattatatataacaatgacaatcactagcgatcgagtagtgagagtcgtcttattacactttcttccttcgatctgtcacatggcggcggcccttatcacttagaagcgtggtgcttcatgtagtagaagtttccgaaaagcatgaggagggtaaccatgtaaacaacgaggagttgagcaatgaacttagggtaaggagaagaagagtagaggaggtaaacagcctggagaaggttcatgaagaactggaacatttgcatctgggtaaggtatcttccccaccaaaggtactttctcttggtcttttcgtccttaggaagaacagcagccatgaagtagtaggtgtacatgcacacatgaacccaagagttgagagcagcagagaagtaagcatctccacctggagcagcataagtgatcatccaccagattccagagatagatccgtggtggtaaacatggaggaaggaaacctggttaacgtttcccttgagaagcatgatgaaggtgtccatgaactcgtagatcttggacacgtagaagatccagatcaccttagccatctcggtttgagcagggttgtaagcgtttccccagaaggagtacttgttcacgtaagcctcgtaaacgagcttgaggcacatgtaaaggctgagtccgataaggaaaacgttgtgagcgagcataagagccttgagaaggaaaggatcctgtcccttaacggttctagggaacactttacggtaaacgagtccagaaccaacgatagcgaagtaagcgaggagagaaaggataagaggggtaggagattcaacgagagggagatccttagtagcagaagagataggcttgagtccccatccaatagagtcggtagcagagaagatagcaggagcaacaacagcatcgatagcagcgtactgctcttgagccatagcaacgagaggttgagcaaattccatggtatggtaattgtaaatgtaattgtaatgttgtttgttgtttgttgttgttggtaattgttgtaaaatgctctgtttgtgtcggaaaataatggaggaagctatgagatgtatttgtatggatcctcttttgtggtccgttacgttttacaaagcatgcatttagacatgtgtatactcaaactcatgcatccatacacattgtaataaagtagtagtccactgaaagttgccaaaatagcaaaatagtacattgcagaaatatatatactaaattcatatatttcgatggaaaatttcggttttccacttaaaataaaatgtacgtataaacttagtcttcttttaacgccaaaaaaaagtctacaaatttctgtctttaatactacattatttttgaattgtgctaaactatgattacatgtgcattaaaatttgagggaatgtgtgttcttagatctgattggcataccctctgactaattatgggatcatgagtatttctcgggaatgtgtttattcgcaagtctattctctaacctcagtaaataatgagtggaagtttagttaaggccaaatagtctaaaatatattatttgtagttttgtacacagccaggattgaatcttaagagactctttaagtctaaaattacaatcagatcctagaccactttctatttgcatgaacgtaaccggatactgattttttaaatgttttctttggttcaaaatcgccactatctttgacaaaaacattctcgaataggattcaaacctaagagcctttcaaattcgttcttaattatgtcatcatctttagttctgctcccatctctcatcggtctcaagaaccactcctagtcatttaagtactacgttttatacacattacatatacatacatttacacaactaggaattgagtagggaacaaagtttcaactttcaactaatagggtaagccttctggtacatggaaaccaaccaaccaatctactagcctgcaggactattttcagaagaagttcccaatagtagtccaaaatttttgtaacgaagggagcataatagttacatgcaaaggaaaactgccattctttagaggggatgcttgtttaagaacaaaaaatatatcactttcttttgttccaagtcattgcgtatttttttaaaaatatttgttccttcgtatatttcgagcttcaatcactttatggttctttgtattctggctttgctgtaaatcgtagctaaccttcttcctagcagaaattattaatacttgggatatttttttagaatcaagtaaattacatattaccaccacatcgagctgcttttaaattcatattacagccatataggcttgattcattttgcaaaatttccaggatattgacaacgttaacttaataatatcttgaaatattaaagctattatgattaggggtgcaaatggaccgagttggttcggtttatatcaaaatcaaaccaaaccaactatatcggtttggattggttcggttttgccgggttttcagcattttctggttttttttttgttagatgaatattattttaatcttactttgtcaaatttttgataagtaaatatatgtgttagtaaaaattaattttttttacaaacatatgatctattaaaatattcttataggagaattttcttaataacacatgatatttatttattttagtcgtttgactaatttttcgttgatgtacactttcaaagttaaccaaatttagtaattaagtataaaaatcaatatgatacctaaataatgatatgttctatttaattttaaattatcgaaatttcacttcaaattcgaaaaagatatataagaattttgatagattttgacatatgaatatggaagaacaaagagattgacgcattttagtaacacttgataagaaagtgatcgtacaaccaattatttaaagttaataaaaatggagcacttcatatttaacgaaatattacatgccagaagagtcgcaaatatttctagatattttttaaagaaaattctataaaaagtcttaaaggcatatatataaaaactatatatttatattttggtttggttcgaatttgttttactcaataccaaactaaattagaccaaatataattgggatttttaatcgagatagaacccacacgagcatgtgctttccatttaattttaaaaaccaagaaacatacatacataacattccatcagcctctctctctttttattacggttaatgacttaaaacacatcttattatcccatccttaacacctagcagtgtctttatacgatctcatcgatcaccacttcaaaaccatgcagactgctgctgcccctggagctggcatcggctaggctgggtgccgcactgtcccggaaggtccctagcgacttgtttagattgatgggaccacctctcaacttcctgctgctgtccctgctgctggatgtcctgcctcatctggccgattgcacgctccagtcccctgcatgtgcactcgctcctcaattgcttaagatcatcgcagcagctatcgaagtgctggctctgttgccctcctccacggccttggttgtagtagtagctgcggcggcccttctggactttttcccacaggaaccgccgaataattcgatagaaccacacgagcatgtgctttcatttattttaaaaaccaagaaacatacataacatttcatcagcctctctctctctctctctctctctctctctctctctctctctctctctctctttattacagctgttacactaacttaaaacacattcatctcattattattattattatccatccttaacacctagcagtgtctttgtacgatctcataatcgatcaccccttcattacttctcagcagctccaactccgcagttgttgatgttacggaacatgagaacaccgttatcaccgtcaacgtattggcaagacctgaaagacttccaaagtgacttccacatgttctcgtcgctagacctgtagtgctttcccataactttcttgatagcctcagaagcaggtctagcgttgtagaatgggatcctagaacagtagtggtgaagcacatgagtctcgatgatatcatggaagatgtgaggtccgatgaatccgaactttctatcgatagtagcagcagcacccttagcgaaagtccattcctcagcgttgtaatgaggcatagtaggatcagtgtgctgaaggaatgtgatgaaaacgagccagtggttaacccagatgtaaggaacgaaccagttgatgaaaagggaccatcctccgaatttcttgtaccaaagagtaagaacgattccctgggtgaggattccaagatcagaaaggaagatgtagagagcatctctttgctcgaaaagtggagaggtaagccagaagtggttccatttccaagaaggaacatcagggtaaggttgtcctgtaacgttaacgaagaggtaagcgatccatcctccaagttgttgaacaagaagctcgtaaagggttctaagtggagaatcctcagagtactcagcgaggttaccgaagaagttcctagacttcttgaattcctctttggtggcaggaacgaaaaccatatctctggtcatgtgtccagtagccttatggtgctttccatgagagtacttccagctgaagtaaggaaccataaggtaagagtgaagggtccatccaacgaaatcgttcacgattccgtaatcagagaaagcttgatgtccacactcatgagcgagaacccagattccggttccgaaaagtccttgaacgtaagtgtaaagggcccagaaagtgaacttgatgatgctgttagaggtgtaagagatgaggagagggtaaaggatcttatgggtaaggtatccggtggtaagcatgcagaagatatctctgaacacgtagtagagagaggtagccaatcttctctcgtaacactcatgagggatagctccaaggatgtccttgatggtgaaatcaggaacagagaacacgtttccgttggtatcgatagcaacttttggaacctcttgctcggtgttgctagaagatcctctgttcttaggatcagatccagtaacggtaacagcgctcatggtatggtaattgtaaatgtaattgtaatgttgtttgttgtttgttgttgttggtaattgttgtaaaatttttggtggtgattggttctttaaggtgtgagagtgagttgtgagttgtgtggtgggtttggtgagattggggatggtgggtttatatagtggagactgaggaatggggtcgtgagtgttaactttgcatgggctacacgtgggttcttttgggcttacacgtagtattattcatgcaaatgcagccaatacatatacggtattttaataatgtgtgggaatacaatatgccgagtattttactaattttggcaatgacaagtgtacatttggattatcttacttggcctctcttgctttaatttggattatttttattctcttaccttggccgttcatattcacatccctaaaggcaagacagaattgaatggtggccaaaaattaaaacgatggatatgacctacatagtgtaggatcaattaacgtcgaaggaaaatactgattctgcccgttcgactcagatcttccaaggcctcgtctccgagtccgctgcttctcgccgcgccgatcacttctccgccgccaacaaggcttgtagttaataggaatcattcagggattgtgattccgggcagtagtaattaataatatagtattagtatagataatatgtttcgtttgggatctttggaacgttgctctgttccttgttgttcattttaaagcttttgagggatagttgcagaactgttcggtgatgcttcatcctctcaagaactagatttgggtaaagaaacatccatgcatggatatggaatgttgttcttccgattggagattattttataaaatttaaaattcatgatttaaaaaaacacataaaaaccacaaaattcatgatttattgacaatacgatacaaaattagcaccaccggctactggctcattacacatttccccttcccctcattctcactttgtggctttattattattattattacatatattttaccgttattatttcacgtcacataagcttgtcattactcagccttagatctaggccttcttccaagagcgtacatatgtctgagggtagaagcaaggttagaccagatagtagggtagtgcttgtactcgattcctctagcctcaagctcagccttaacaagaggagcaagtctagggtagaatccatggtgaactctagggaacaagtgatgctcaatttggtagttgagtccaccgttaagagtagcaagaagaggtcctccaacgttagaagaagtctcagcttgtctcttaaggaagctagcacctctagtcatagaagtgatagatccatcaggtccaacagaagcaacaccctcgaagttgtgggagatgaagaagaagaaagcgaggtagaaagatccagtcataacagtagcagcgatacacacagcagtatgaacagaaggagcaaggtaaagaggcaaagcaacgaatctagcccagaaggtaagcttgagaagcaaagaaggcataaagaggtatccagcaagcttagagataggctcaccctcccaacgccacataacaagctcagagatgtcgaggaacaaaagcttgaaagcgtacatagtctcaccaggcaaaaggtaaagatgctgaagccaatgcataggtgaccaagcatcagtaggcttgagtctaagagcaccgtgagccttttgatcaggatccttatcaacatcgttagtgtggaggtggtgcataacaacatgctcttgaagccaaaggatcatagatcctccgatccaatcctgacaaagtccaagagcaaggttaacagaagcagacttagacaaagcaccatggttagcatcatgctggatgttaagaccgataagagcgaaaagccatccaagaacgatagaagggagaagtctctttccagcgtaaagcatgtaagcctcaagagcgatagcagatccaaggataagtccagccttaacccagtaagaagcaggagcgaatccagaagaaacagaaggcaccatcttagcgatcctagcacaaagttgaaggtatccctcatcagcagcaacaggttcctcagtagaagcaagagatccaacgtggaatctagacattctagacttaggccaagcccttctatggtattccatgaaagcctcagtagcatctcttcctccgaacaaagaaacgaaatgagcaccaccaggatgctcagatctgaaagccttagcatcgtaaacagaatctccaacgatggtgagatcaggtctatcagcaacatcctttctggtgaaagcagaagagtcagtaacaccagcatgaacaccagtagaagctcccatttgcttagcagcgctaggtggcatggtatggtaattgtaaatgtaattgtaatgttgtttgttgtttgttgttgttggtaattgttgtaaaagtgggtatcttttggatggataagcaagtagtgatgatgttctaggtgaagtgatgggggtgttttatagcgggagatggtgaaatggatggtcgccacataagaaatggaggggaagggttcttgcgccattcttcagtttgcatggatgcatgggtttcattttgtaacacgtaataaggacaatgaagtgcaggtgtctctcaagtttcagaggggatatgtggacagaagaagaacggcgatgatattgatggaaatggccatctagtgtgaatctattcggttgataatactagtgcattttggccgttaatcccttcaattaactgcacaaacttcagttgagtattgattatttgattataggttctgtaaacacaataccaagtttatttagaggggagacatacaaatagtttcgatataaataatagagtggttaaacttagttattaaaactatatataaagtctaaaagttaaattatttttttaattgcaaatatataaagtctaaaggggttacattatttcttaagagatgtaactctgttggaatctgacttaatccgtctcatcactctggtttccagttctaatctaatgaattgttttctgccaaagaatttgaagcaagaagtaaattgatcaatgccgtcaacccacaccaaaccgtcaacccactaccatcgccgcggagacccccaaactcaacctccacccatcggtaagaagcacagggcagcccgcaccaccaccaatttggcgtgcatgacacctagggacttggcacgggaggcggcgcacgtggatgcaaatgacgggatatcagatgacaggaaacgacgttgagagaccatacgatgtagaatatgagctcaccatcaacgagaaactaggaaaatcacaaaaaaaacaactctcgtaattgtacgagtggcacagatgggtctgcctcaacatatctctaatacggcgaagcctgcccaacacgtagttgccggaatccggtgtggagctcacgactctgaaagataggcgcttcctgtttcgtttcgctcacccactggacgtccgtcatgtgatggatttcggtcattggtttgctgacaaccacattctgaagctccatgagatgagtcttcacaataggtcctgctcaataccgtggagttatggttgcaagtccataacttgccgttcgaatattttgcggagccagtcggacgggaattggcgagctcggctgacacctataaaggccatgacaagaagaaccaaaagttcttccctaatgctttcatgaggcttcgggtcgttatggatgtcggaaaacccctcttgaaggaacgagacgttattatgcatgacggtaagactattacttgtcagtataagtatgaaagattacctgtcttctgctttgtttgtggattgattggacacgttgaaaaaaaatgtgcacttcgatttcaatactcagagatcgacttcccttttctctaggagtattcgatcaaggcattaacatggaaggaagctcaagctctaaaggcttcacaatggaacctgaaaaatttcaacaagcctaaactgaaatcgaagtcaaatcacccaaccgggagctctaaatcagcaaacactcctcctccacagtatccaatcatcgtgcacgatgctccaggtattgcaagccaggtattgcaagctaggagtaggatagagaccttaaacgtcgttggtgtgaagagtcatcttcagacctaatggagatagatgtagacggcggcacgaagactctgaaacaccagaaaggctagtccaggataaggatctgctatcccaactgacctctcgttagtcccaaggcctctcaactagagcaggaggaaggatggtcacaagactaggataatgatgtttccaatatgaacctgaatgtccatagctaatttttttagtcttgcttctgcactttttgtttattatgttctggtgactatgttatttacccttgtccgtatgcttgagagaatcagtattttccttcgacgttaattgatcctacactatgtaggtcatatccatcgttttaatttttggccaccattcaattctgtcttgcctttagggatgtgaatatgaacggccaaggtaagagaataaaaataatccaaattaaagcaagagaggccaagtaagataatccaaatgtacacttgtcattgccaaaattagtaaaatactcggcatattgtattcccacacattattaaaataccgtatatgtattggctgcatttgcatgaataatactacgtgtaagcccaaaagaacccacgtgtagcccatgcaaagttaacactcacgaccccattcctcagtctccactatataaacccaccatccccaatctcaccaaacccaccacacaactcacaactcactctcacaccttaaagaaccaatcaccaccaaaaattttacaacaattaccaacaacaacaaacaacaaacaacattacaattacatttacaattaccataccatgtctaaggttaccgtgtctggatctgagatccttgagggatctactaagaccgttaggcgttctggaaacgttgcatctttcaagcagcaaaagaccgctatcgataccttcggaaacgttttcaaggtgccagattacaccatcaaggatatccttgacgctatccctaagcactgttacgagagatctctcgtgaagtctatgtcttacgtggtgagagatatcgtggctatctctgctatcgcttacgttggacttacctacatccctcttctccctaacgaattccttagattcgctgcttggtctgcttacgtgttctctatctcttgtttcggattcggaatctggatccttggacatgagtgtggacattctgctttctctaactacggatgggttaacgataccgttggatgggttctccactctcttgttatggttccttacttcagctggaagttctctcatgctaagcaccataaggctactggacacatgaccagagatatggttttcgttccttacaccgccgaggaattcaaagagaagcaccaagttaccagccttcacgatatcgctgaggaaactcctatctactctgttttcgctctcttgttccaacagcttggaggactttctctttaccttgctactaacgctactggacaaccttaccctggtgtttctaagttcttcaagtctcactactggccttctagccctgttttcgataagaaggactactggtacatcgttctttctgatcttggaatccttgctaccctcacttctgtttacaccgcttacaaggttttcggattctggcctactttcatcacatggttctgtccttggatccttgttaaccactggcttgttttcgttaccttccttcagcacaccgattcttctatgcctcattacgatgctcaagagtggactttcgctaagggtgctgctgctactatcgatagagagttcggaatcctcggaatcatcttccatgacatcatcgagactcatgtgctccatcactacgtttcaaggatcccattctaccatgctagagaagctaccgagtgcatcaagaaagttatgggagagcactacagacacaccgatgagaacatgtgggttagcctttggaaaacttggagatcttgccagttcgttgagaaccatgatggtgtgtacatgttccgtaactgcaacaacgttggagtgaagcctaaggatacctgatgaaggggtgatcgattatgagatcgtacaaagacactgctaggtgttaaggatggataataataataataatgagatgaatgtgttttaagttagtgtaacagctgtaataaagagagagagagagagagagagagagagagagagagagagagagagagagaggctgatgaaatgttatgtatgtttcttggtttttaaaataaatgaaagcacatgctcgtgtggttctatcgaattattcggcggttcctgtgggaaaaagtccagaagggcggcggcagctactactacaaccaaggccgtggaggagggcaacagagccagcacttcgatagctgctgcgatgatcttaagcaattgaggagcgagtgcacatgcaggggactggagcgtgcaatcggccagatgaggcaggacatccagcagcagggacagcagcaggaagttgagaggtggtcccatcaatctaaacaagtcgctagggaccttccgggacagtgcggcacccagcctagccgatgccagctccaggggcagcagcagtctgcatggttttgaagtggtgatcgatgagatcgtataaagacactgctaggtgttaaggatgggataataagatgtgttttaagtcattaaccgtaataaaaagagagagaggctgatggaatgttatgtatgtatgtttcttggtttttaaaattaaatggaaagcacatgctcgtgtgggttctatcactattttcagaagaagttcccaatagtagtccaaaatttttgtaacgaagggagcataatagttacatgcaaaggaaaactgccattctttagaggggatgcttgtttaagaacaaaaaatatatcactttcttttgttccaagtcattgcgtatttttttaaaaatatttgttccttcgtatatttcgagcttcaatcactttatggttctttgtattctggctttgctgtaaatcgtagctaaccttcttcctagcagaaattattaatacttgggatatttttttagaatcaagtaaattacatattaccaccacatcgagctgcttttaaattcatattacagccatataggcttgattcattttgcaaaatttccaggatattgacaacgttaacttaataatatcttgaaatattaaagctattatgattaggggtgcaaatggaccgagttggttcggtttatatcaaaatcaaaccaaaccaactatatcggtttggattggttcggttttgccgggttttcagcattttctggttttttttttgttagatgaatattattttaatcttactttgtcaaatttttgataagtaaatatatgtgttagtaaaaattaattttttttacaaacatatgatctattaaaatattcttataggagaattttcttaataacacatgatatttatttattttagtcgtttgactaatttttcgttgatgtacactttcaaagttaaccaaatttagtaattaagtataaaaatcaatatgatacctaaataatgatatgttctatttaattttaaattatcgaaatttcacttcaaattcgaaaaagatatataagaattttgatagattttgacatatgaatatggaagaacaaagagattgacgcattttagtaacacttgataagaaagtgatcgtacaaccaattatttaaagttaataaaaatggagcacttcatatttaacgaaatattacatgccagaagagtcgcaaatatttctagatattttttaaagaaaattctataaaaagtcttaaaggcatatatataaaaactatatatttatattttggtttggttcgaatttgttttactcaataccaaactaaattagaccaaatataattgggatttttaatcgaccgatctagtaacatagatgacaccgcgcgcgataatttatcctagtttgcgcgctatattttgttttctatcgcgtattaaatgtataattgcgggactctaatcataaaaacccatctcataaataacgtcatgcattacatgttaattattacgtgcttaacgtaattcaacagaaattatatgataatcatcgcaagaccggcaacaggattcaatcttaagaaactttattgccaaatgtttgaacgatctcattactgcattttcttctcaggagcatgggcaacgttatcaaggttagcgaaagtatcagccatagcctcgaagtatcctctaacatcgtagtgaagtccgtgcttctcgaaaagctgcttaactctaggagcgatcttagggtgtctgaattgaggcatagaagggtaaaggtggtgctcgatctggtagttaaggtaagacatccaccaatcacaccaccaagatggagaacagttagtagtgtggttagcagcgtactcaacccaagtagcatgctcgttaggctcaacaacagggaggtgagtatgagaaacagcgaagttgcagaagatgtacatagctccaagctgaacgtaaagaaggtaacaagcgagaacgtatccagcaccgtagttagcagcaaggtatccaacaagtccgtatctgattccgagcatagcaagctcatcgtagtgcttagtcctgagcatgtgtctaggatgaaggtaaagctgccatccaagagcaacaagaagagtggtaacaggagcgaaaagcttagcttgcatagaaagccaagccttcatagcaggagacttaaccttagcagcgattctctcatggaaagcaacgagaggaagggtatcaagatcaacatcgtgctgaagcttttgaggagtagcatggtgcttgttatgctggttacgccaccaagcaccagacattccacatccaagtccgtaacaagcaacttggatagctctgtcgaaagcaatgtttccagtgagagagtaatgtccaccctcatgcataagccatccacatcttccctgaacaactccaagcatagcgattccagcgaaagtgtatccatgccagataagagcagcaccagcaacatgcatagcgataacctcagcaagtctgtaagcaacatgaggaagagaaggctcgaacattccctcagcctcaagttgcttggtgaactcttggaaatcagcgataagatcagcccttcttggagagtatcccttgtgaacaggacgagaaggaagagacttaagcatcttgtcagccttagcagatctaacatggaactgcttgtaagcatcggtagcatcagttccaacttggtaagcaatgatctttccaccagggtgtctcttaacgaagttggtaacatcgtaagccctatctccgataacaagctctttcttgtcgtgctcttgaggagtatcaacttcgtgaagttgagcagaaggaggagcagcataagagtaagagtcccttggaggcatggtatggtaattgtaaatgtaattgtaatgttgtttgttgtttgttgttgttggtaattgttgtaaaagatcctcgtgtatgtttttaatcttgtttgtatcgatgagttttggtttgagtaaagagtgaagcggatgagttaatttataggctataaaggagatttgcatggcgatcacgtgtaataatgcatgcacgcatgtgattgtatgtgtgtgctgtgagagagaagctcttaggtgtttgaagggagtgacaagtggcgaagaaaaacaattctccgcggctgcatgctatgtgtaacgtgtagctaatgttctggcatggcatcttatgaacgattctttttaaaaacaaggtaaaaacttaacttcataaaattaaaaaaaaaaacgtttactaagttggtttaaaaggggatgagactagaatctaattattctattcagactaaattagtataagtatttttttaatcaataaataataattaataatttattagtaggagtgattgaatttataatatattttttttaatcatttaaagaatcttatatctttaaattgacaagagttttaaatggggagagtgttatcatatgacaagtaggattaatgtgttatagtttcacatgcattacgataagttgtgaaagataacattattatatataacaatgacaatcactagcgatcgagtagtgagagtcgtcttattacactttcttccttcgatctgtcacatggcggcggcccggcgcgccgcgcgccttatcactgcttcttagcacccttagacttgtacctcttacggtagaagttggcgaagagaacgaacatgttcaccataacccagagttgaaggtaaggaagccagaaagcggtattctgaacgtaagcggtgtagatagagtgagaagcacagatacagaactgaagcatctggatctgggtgatgtacttcttccagaaacagttaactccaagagcagcaagtccgtagtaagagtacatgatcacgtgcacgaaggtgttaacagaagatccgaagtagcaatctccaacaggctcaagcttcataacaacgaaccatgaccagatgagaagagtgtggtggtagatgtgaaggaaagaaagctggtcgaacttcttcctcatcaccatgaagaaggtgtcgagaagctcaacgtacttgttgttgtagtgaagccagataacctgagagattccccaagagttagcagtcatatcagggatgtttccccaaaccttaagtccctgagccctatgagaagtaacgaaaaggtagatgcagtagctgttgaagaaggtctggtagaagttgtaaacgagcatagcgttcttgagtccgaaaggttgagatctgttctgcatgatacgctttccgaagtagatgaagaggaggtatccaatagttccgatagtaggtccccagtactcaacctgcatgaagtaagcaggaactttctcagaagctgggatatcagggttagccacattgtaggtaacgtatccaagagttccagcaagagcagcagggatagcgatagaggccatggtatggtaattgtaaatgtaattgtaatgttgtttgttgtttgttgttgttggtaattgttgtaaaatgctctgtttgtgtcggaaaataatggaggaagctatgagatgtatttgtatggatcctcttttgtggtccgttacgttttacaaagcatgcatttagacatgtgtatactcaaactcatgcatccatacacattgtaataaagtagtagtccactgaaagttgccaaaatagcaaaatagtacattgcagaaatatatatactaaattcatatatttcgatggaaaatttcggttttccacttaaaataaaatgtacgtataaacttagtcttcttttaacgccaaaaaaaagtctacaaatttctgtctttaatactacattatttttgaattgtgctaaactatgattacatgtgcattaaaatttgagggaatgtgtgttcttagatctgattggcataccctctgactaattatgggatcatgagtatttctcgggaatgtgtttattcgcaagtctattctctaacctcagtaaataatgagtggaagtttagttaaggccaaatagtctaaaatatattatttgtagttttgtacacagccaggattgaatcttaagagactctttaagtctaaaattacaatcagatcctagaccactttctatttgcatgaacgtaaccggatactgattttttaaatgttttctttggttcaaaatcgccactatctttgacaaaaacattctcgaataggattcaaacctaagagcctttcaaattcgttcttaattatgtcatcatctttagttctgctcccatctctcatcggtctcaagaaccactcctagtcatttaagtactacgttttatacacattacatatacatacatttacacaactaggaattgagtagggaacaaagtttcaactttcaactaatagggtaagccttctggtacatggaaaccaaccaaccaatctactagggtaccctcaagcatacggacaagggtaaataacatagtcaccagaacataataaacaaaaagtgcagaagcaagactaaaaaaattagctatggacattcaggttcatattggaaacatcattatcctagtcttgtgaccatccttcctcctgctctagttgagaggccttgggactaacgagaggtcagttgggatagcagatccttatcctggactagcctttctggtgtttcagagtcttcgtgccgccgtctacatctatctccattaggtctgaagatgactcttcacaccaacgacgtttaaggtctctatcctactcctagcttgcaatacctggcttgcaatacctggagcatcgtgcacgatgattggatactgtggaggaggagtgtttgctgatttagagctcccggttgggtgatttgacttcgatttcagtttaggcttgttgaaatttttcaggttccattgtgaagcctttagagcttgagcttccttccatgttaatgccttgatcgaatactcctagagaaaagggaagtcgatctctgagtattgaaatcgaagtgcacattttttttcaacgtgtccaatcaatccacaaacaaagcagaagacaggtaatctttcatacttatactgacaagtaatagtcttaccgtcatgcataataacgtctcgttccttcaagaggggttttccgacatccataacgacccgaagcctcatgaaagcattagggaagaacttttggttcttcttgtcatggcctttataggtgtcagccgagctcgccaattcccgtccgactggctccgcaaaatattcgaacggcaagttatggacttgcaaccataactccacggtattgagcaggacctattgtgaagactcatctcatggagcttcagaatgtggttgtcagcaaaccaatgaccgaaatccatcacatgacggacgtccagtgggtgagcgaaacgaaacaggaagcgcctatctttcagagtcgtgagctccacaccggattccggcaactacgtgttgggcaggcttcgccgtattagagatatgttgaggcagacccatctgtgccactcgtacaattacgagagttgttttttttgtgattttcctagtttctcgttgatggtgagctcatattctacatcgtatggtctctcaacgtcgtttcctgtcatctgatatcccgtcatttgcatccacgtgcgccgcctcccgtgccaagtccctaggtgtcatgcacgccaaattggtggtggtgcgggctgccctgtgcttcttaccgatgggtggaggttgagtttgggggtctccgcggcgatggtagtgggttgacggtttggtgtgggttgacggcattgatcaatttacttcttgcttcaaattctttggcagaaaacaattcattagattagaactggaaaccagagtgatgagacggattaagtcagattccaacagagttacatctcttaagaaataatgtaacccctttagactttatatatttgcaattaaaaaaataatttaacttttagactttatatatagttttaataactaagtttaaccactctattatttatatcgaaactatttgtatgtctcccctctaaataaacttggtattgtgtttacagaacctataatcaaataatcaatactcaactgaagtttgtgcagttaattgaagggattaacggccaaaatgcactagtattatcaaccgaatagattcacactagatggccatttccatcaatatcatcgccgttcttcttctgtccacatatcccctctgaaacttgagagacacctgcacttcattgtccttattacgtgttacaaaatgaaacccatgcatccatgcaaactgaagaatggcgcaagaacccttcccctccatttcttatgtggcgaccatccatttcaccatctcccgctataaaacacccccatcacttcacctagaacatcatcactacttgcttatccatccaaaagatacccacttaattaattttacaacaattaccaacaacaacaaacaacaaacaacattacaattacatttacaattaccataccatgtgccctcctaagactgatggaagatcttctcctagatctccacttaccaggtctaaatcttctgctgaggctcttgatgctaaggatgcttctactgctcctgttgatcttaagactcttgagcctcatgagcttgctgctactttcgagactagatgggttagagttgaggacgttgagtacgatgtgactaacttcaagcaccctggtggatctgtgatcttctacatgcttgctaacactggtgctgatgctactgaggctttcaaagaattccacatgcgttctctcaaggcttggaagatgcttagagctttgccttctagacctgctgagatcaagagatctgagtctgaggatgctcctatgcttgaggatttcgctagatggcgtgctgagcttgagagagatggattcttcaagccttctatcacccatgtggcttacagacttctcgagcttcttgctacattcgctcttggaactgctcttatgtacgctggataccctatcattgcttctgttgtttacggtgctttcttcggagctagatgtggatgggttcaacatgagggtggacataactctcttaccggatctgtttacgtggacaagagacttcaggctatgacttgtggattcggactttctacttctggtgagatgtggaaccagatgcataacaagcaccatgctacccctcaaaaggttagacacgatatggatcttgataccactcctgctgtggctttcttcaacactgctgttgaggataacagacctagaggattctctagagcttgggctagacttcaagcttggactttcgttcctgttacctctggacttcttgttcaagctttctggatctacgttctccaccctagacaagttctccgtaagaagaactacgaagaggcttcttggatgctcgtttctcatgttgttagaaccgctgttatcaagcttgctactggatactcttggcctgttgcttactggtggttcactttcggaaactggatcgcttacatgtaccttttcgctcacttctctacttctcatactcacctccctgttgttccatctgataagcacctttcttgggttaactacgctgttgatcacaccgttgatatcgatccttctagaggatacgtgaactggcttatgggataccttaactgtcaggttatccaccacctcttccctgatatgcctcaattcagacagcctgaggttagcagaagattcgttcctttcgctaagaagtggggactcaactacaaggtgctctcttactacggtgcttggaaggctactttctctaaccttgataaggtgggacagcactactacgttaacggaaaggctgagaaggctcactaatgattaattaacaagcttatgtgacgtgaaataataacggtaaaatatatgtaataataataataataaagccacaaagtgagaatgaggggaaggggaaatgtgtaatgagccagtagccggtggtgctaattttgtatcgtattgtcaataaatcatgaattttgtggtttttatgtgtttttttaaatcatgaattttaaattttataaaataatctccaatcggaagaacaacattccatatccatgcatggatgtttctttacccaaatctagttcttgagaggatgaagcatcaccgaacagttctgcaactatccctcaaaagctttaaaatgaacaacaaggaacagagcaacgttccaaagatcccaaacgaaacatattatctatactaatactatattattaattactactgcccggaatcacaatccctgaatgattcctattaactacaagccttgttggcggcggagaagtgatcggcgcggcgagaagcagcggactcggagacgaggccttggaagatctgagtcgaacgggcggtaccgcggccgcaagctttccgcggggcgcccgttttacaacgtcgtgactgggagatccactagcagattgtcgtttcccgccttcagtttaaactatcagtgtttgaaggacagacccacccaagaacacaccagtcattcagatgcagcctatctccgtgccggctattccagctgatgagttgaaggatataactgataactatggttccaagtccttgattggtgagggctcttatggaagagtgttttacggtgttcttagaagcggcaaggcagctgccattaagaagctggattctagtaagcagcctgatcaagagtttctcgcacaggtacaaatgctacttaagtaaatcaaaccgttaaagttgagttgctgcttagttactgatgtaaataatgttaattaggtatcaatggtttcgagattgagacaagacaatgttgttgcacttctgggatattgcgttgatggcccactccgtgttcttgcttatgagtttgctcctaatggatctcttcatgatattcttcatggtaagttattaagtctaaaacattgattcggtacgacttgtagatgtgaagctattaactaatgaaatgtggtgagtttgttgggtgtaggtaggaaaggagtgaaaggagcacagccaggacctgttctgtcgtggaaccagagagttaaaattgctgttggtgcggctaggggactcgagtacttgcatgagaaggcgaaccctcatgttgtccaccgagacatcaaatccagcaatgtgcttttgtttgacgatgatgttgccaagattgctgacttcgatctgtctaaccaagcccctgacatggctgctcgccttcactcaactcgtgtgctgggaacctttggttatcacgctccagagtaagccctttacttgtttatttgaattgtttttgttcagactaatcaatgtggttacattcaacttgtgctcaaagacttttggttattattatcttatgttttgaggcactaagtccttccttggaataatctttgacattattttggattgcatctcttctaattgaccatactagagtcttaaacacaaacatttttgttttggttctgcattttcaggtatgcaatgacagggacattgagcacaaagagtgatgtctatagttttggagttgttctgctagagctcctcacaggtcgtaagccagttgatcataccttaccacgaggacagcagagtctcgttacatgggtaatgcttagtgcagctctgcttcttttttctggtttactcatattgagaagaaaagggaatgtgtctgcacaatcatgttgattttgtgagagattagataaactcattattaaatgaaaacgcgtttgtgtgtgtgtatcaggcaactcctaaactgagtgaagacaaggtgaagcaatgcgttgatgcaagactaaacggagaatatcctcccaaagctgttgccaaggtaaccttttgtcatagtgtcgttgtgtcagtagagaaggtttaccttaggacacgacttagaaactgcttctccatcacttccatcgttttcggttccttcttaatgtatccctgttgtaggcctagattgaaatacaagtctcttctaaggacaatagaacctaagcattgatgtatgatttttttgggagtctgattttggttttttctctcttatatgactccggtaatgatcagctggctgctgtagctgcgctatgtgtgcaatacgaagcagacttcaggccaaacatgagcatagtggtgaaggctcttcagcctctcctcaatcctcctcgctctgctcctcaaactcctcacaggaacaatccttattgatgtcctccaatctgatgccacgcttcttcatcatatcacttatttcatttgtttttgtttgaatccaatttgtgtaaattcgtgaaaataggctttttatttctcacaatagacatgaaagtctcacttccaaacctgaatggtgttgctctatttgtttatgttatttcatgcctgcgattgtaagtttctactaattatacaatatgcgaggaatggattattcataatatactcattgtgtttgtgcc

SEQ ID NO: 42 - DNA, 18 bp, synthetic construct
  misc_feature 1..18: note = Junction at 5' end of transgene
  source 1..18: mol_type = other DNA
tggaggtgttcaaacact

SEQ ID NO: 43 - DNA, 18 bp, synthetic construct
  misc_feature 1..18: note = Junction of 5' end of 4-transgene-insert on chr. A02.
  source 1..18: mol_type = other DNA
tggaggtgttcaaacact

SEQ ID NO: 44 - DNA, 18 bp, synthetic construct
  misc_feature 1..18: note = Junction of 3' end of 4-trangene-insert and chr. A02
  source 1..18: mol_type = other DNA
atagtattagtatacaga

SEQ ID NO: 45 - DNA, 18 bp, synthetic construct
  misc_feature 1..18: note = Junction of 5' end of 16-transgene insert in chr. A05
  source 1..18: mol_type = other DNA
ggctaaggtaacactgat

SEQ ID NO: 46 - DNA, 18 bp, synthetic construct
  misc_feature 1..18: note = Junction of 3' end of 16-transgene insert and chr. A05
  source 1..18: mol_type = other DNA
cagtgtttgaaggacaga

SEQ ID NO: 47 - DNA, 470 bp, synthetic construct
  misc_feature 1..470: note = 470 bp chimeric 5' junction of transgenic insert and Brassica chr. A02
  source 1..470: mol_type = other DNA
cattgagcagtgaacaccaaggataaatatttactgattagtgtgtgattgaatcaaagaaaggttagaatctggttttcatttagccattcaatctcgatgtaaaatcggttagattctggttgttgatacttgagaacttgaaatgttttgtaactgtgaattttgttttgaaaatagacaagtgaatctgtttggggttgtgtgaaaacgtgtgagcaattgttggaggtgttcaaacactgatagtttaaactgaaggcgggaaacgacaatctgctagtggatctcccagtcacgacgttgtaaaacgggcgccccgcggaaagcttgcggccgcggtaccgcccgttcgactcagatcttccaaggcctcgtctccgagtccgctgcttctcgccgcgccgatcacttctccgccgccaacaaggcttgtagttaataggaatcattcagggattgtgattccg

SEQ ID NO: 48 - DNA, 470 bp, synthetic construct
  misc_feature 1..470: note = 470 bp chimeric 3' junction of transgenic insert and Brassica chr. A02
  source 1..470: mol_type = other DNA
ttgaatggtggccaaaaattaaaacgatggatatgacctacatagtgtaggatcaattaacgtcgaaggaaaatactgattctgcccgttcgactcagatcttccaaggcctcgtctccgagtccgctgcttctcgccgcgccgatcacttctccgccgccaacaaggcttgtagttaataggaatcattcagggattgtgattccgggcagtagtaattaataatatagtattagtatacagaacctcttatttagctaaaagattatgttcttaatgttgataagaagtttgagaaacaaatataattgagcttctgattagttgatcgtaattggtcattaataattgtatctaaccagtgcagtataagagcgtataagagcatcttcaaaaagactttattttagagttaatcagtgcagtataagagcatctctaaaaaaactctaattatagagttttgcaaa

SEQ ID NO: 49 - DNA, 470 bp, synthetic construct
  misc_feature 1..470: note = 470 bp chimeric 5' junction of transgene insert and chr. A05
  source 1..470: mol_type = other DNA
cttgttccgcaacaccgttactgaactcttcgttcacttaaacagtttgtgtgtgtgagaaacagcgtaatgagctgctttggttgttgtggtggtgacgattttcgtcgagttgctgaaactggacccaagccagtgtacggcgcaggaggtactttaagcttataaccctttgtctatcctttggctagcggctaatgttgatgaacttttttattcaaccgttggctaaggtaacactgatagtttaaactgaaggcgggaaacgacaatctgctagtggatctcccagtcacgacgttgtaaaacgggcgccccgcggaaagcttgcggccgcggtaccgcccgttcgactcagatcttccaaggcctcgtctccgagtccgctgcttctcgccgcgccgatcacttctccgccgccaacaaggcttgtagttaataggaatcattcagggattgtgattccgggc

SEQ ID NO: 50 - DNA, 470 bp, synthetic construct
  misc_feature 1..470: note = 470 bp chimeric 3' junction of transgene insert and chr. A05
  source 1..470: mol_type = other DNA
ccggaatcacaatccctgaatgattcctattaactacaagccttgttggcggcggagaagtgatcggcgcggcgagaagcagcggactcggagacgaggccttggaagatctgagtcgaacgggcggtaccgcggccgcaagctttccgcggggcgcccgttttacaacgtcgtgactgggagatccactagcagattgtcgtttcccgccttcagtttaaactatcagtgtttgaaggacagacccacccaagaacacaccagtcattcagatgcagcctatctccgtgccggctattccagctgatgagttgaaggatataactgataactatggttccaagtccttgattggtgagggctcttatggaagagtgttttacggtgttcttagaagcggcaaggcagctgccattaagaagctggattctagtaagcagcctgatcaagagtttctcgcacaggtacaa

SEQ ID NO: 51 - DNA, 24 bp, synthetic construct
  misc_feature 1..24: note = Forward primer for amplicon diagnostic for NS-B50027-4
  source 1..24: mol_type = other DNA
aattgttggaggtgttcaaacact

SEQ ID NO: 52 - DNA, 24 bp, synthetic construct
  misc_feature 1..24: note = Reverse primer for amplicon diagnostic for NS-B50027-4
  source 1..24: mol_type = other DNA
cggaatcacaatccctgaatgatt

SEQ ID NO: 53 - DNA, 20 bp, synthetic construct
  misc_feature 1..20: note = Sense primer for detection of codon-optimized delta12-desaturase
  source 1..20: mol_type = other DNA
tggagctatccctcatgagt

SEQ ID NO: 54 - DNA, 21 bp, synthetic construct
  misc_feature 1..21: note = Antisense primer for detection of codon-optimized delta12-desaturase
  source 1..21: mol_type = other DNA
gatcctagaacagtagtggtg

SEQ ID NO: 55 - DNA, 21 bp, synthetic construct
  misc_feature 1..21: note = Sense primer for detecting codon-optimized delta15/omega3-desaturase
  source 1..21: mol_type = other DNA
gacgctatccctaagcactgt

SEQ ID NO: 56 - DNA, 20 bp, synthetic construct
  misc_feature 1..20: note = Antisense primer for detecting codon-optimized delta15/omega3-desaturase
  source 1..20: mol_type = other DNA
gtccactcttgagcatcgta

SEQ ID NO: 57 - DNA, 21 bp, synthetic construct
  misc_feature 1..21: note = Sense primer for detecting codon-optimized delta6-desaturase
  source 1..21: mol_type = other DNA
gagcaccttgtagttgagtcc

SEQ ID NO: 58 - DNA, 21 bp, synthetic construct
  misc_feature 1..21: note = Antisense primer for detecting codon-optimized delta6-desaturase
  source 1..21: mol_type = other DNA
agtctgaggatgctcctatgc

SEQ ID NO: 59 - DNA, 20 bp, synthetic construct
  misc_feature 1..20: note = Sense primer for detecting codon-optimized delta6-elongase
  source 1..20: mol_type = other DNA
tgttgctatggctcaagagc

SEQ ID NO: 60 - DNA, 20 bp, synthetic construct
  misc_feature 1..20: note = Antisense prmer for detecting codon-optimized delta6-elongase
  source 1..20: mol_type = other DNA
ctagcgtggtgcttcatgta

SEQ ID NO: 61 - DNA, 20 bp, synthetic construct
  misc_feature 1..20: note = Sense primer for detection codon-optimized delta5-desaturase
  source 1..20: mol_type = other DNA
gctaccgatgcttacaagca

SEQ ID NO: 62 - DNA, 20 bp, synthetic construct
  misc_feature 1..20: note = Antisense primer for detecting codon-optimized delta5-desaturase
  source 1..20: mol_type = other DNA
tagtgaagtccgtgcttctc

SEQ ID NO: 63 - DNA, 20 bp, synthetic construct
  misc_feature 1..20: note = Sense primer for detection of delta5-elongase
  source 1..20: mol_type = other DNA
tgctggaactcttggatacg

SEQ ID NO: 64 - DNA, 20 bp, synthetic construct
  misc_feature 1..20: note = Antisense primer for detection of codon-optimized delta5-elongase
  source 1..20: mol_type = other DNA
ctgggtgatgtacttcttcc

SEQ ID NO: 65 - DNA, 20 bp, synthetic construct
  misc_feature 1..20: note = Sense primer for detecting codon-optimized delta4-desaturase
  source 1..20: mol_type = other DNA
ggctttcagatctgagcatc

SEQ ID NO: 66 - DNA, 20 bp, synthetic construct
  misc_feature 1..20: note = Antisense primer for detecting codon-optimized delta4-desaturase
  source 1..20: mol_type = other DNA
ctcagccttaacaagaggag